European Patent Specification EP 3 802 598 B1, published February 12, 2025. Title: Multi-specific binding proteins for cancer treatment. Applicant: Boehringer Ingelheim International GmbH. The sequence listing filed with the application follows.

SEQUENCE LISTING (265 sequences)

SEQ ID NO: 1 - protein, 12 aa, Artificial Sequence
  DLL3# 1LCCDR1
RASQSVSSNFLV

SEQ ID NO: 2 - protein, 7 aa, Artificial Sequence
  DLL3#1 LCCDR2
GASTRAS

SEQ ID NO: 3 - protein, 9 aa, Artificial Sequence
  DLL3#1 LCCDR3
QQYGDSPYT

SEQ ID NO: 4 - protein, 10 aa, Artificial Sequence
  DLL3#1 HCCDR1
GNTFTNYYMH

SEQ ID NO: 5 - protein, 17 aa, Artificial Sequence
  DLL3#1 HCCDR2
IIDPSVGSKSYAQKFLG

SEQ ID NO: 6 - protein, 12 aa, Artificial Sequence
  DLL3#1 HCCDR3
AGKRFGESYFDY

SEQ ID NO: 7 - protein, 11 aa, Artificial Sequence
  DLL3#2 LCCDR1
RASQGISNYLA

SEQ ID NO: 8 - protein, 7 aa, Artificial Sequence
  DLL3#2 LCCDR1
AASSLQS

SEQ ID NO: 9 - protein, 9 aa, Artificial Sequence
  DLL3#2 LCCDR1
LQHNSSPYT

SEQ ID NO: 10 - protein, 10 aa, Artificial Sequence
  DLL3#2 HCCDR1
GYTFTSYYMH

SEQ ID NO: 11 - protein, 17 aa, Artificial Sequence
  DLL3#2 HCCDR2
IINPSGGSTSYAQKFQG

SEQ ID NO: 12 - protein, 15 aa, Artificial Sequence
  DLL3#2 HCCDR3
GEAVGGNYYYYGMDV

SEQ ID NO: 13 - protein, 11 aa, Artificial Sequence
  DLL3#3 LCCDR1
RASQGISNYLV

SEQ ID NO: 14 - protein, 7 aa, Artificial Sequence
  DLL3#3 LCCDR2
AVSSLYS

SEQ ID NO: 15 - protein, 9 aa, Artificial Sequence
  DLL3#3 LCCDR3
LQHDSYPYT

SEQ ID NO: 16 - protein, 10 aa, Artificial Sequence
  DLL3#3 HCCDR1
GYTFTSYYVH

SEQ ID NO: 17 - protein, 17 aa, Artificial Sequence
  DLL3#3 HCCDR2
IINPGGGTTSYAQKFLG

SEQ ID NO: 18 - protein, 15 aa, Artificial Sequence
  DLL3#3 HCCDR3
GEAVTGNYFYYGMDV

SEQ ID NO: 19 - protein, 15 aa, Artificial Sequence
  DLL3#4 LCCDR1
RASKSVSSFGYSFMH

SEQ ID NO: 20 - protein, 7 aa, Artificial Sequence
  DLL3#4 LCCDR2
LASNLES

SEQ ID NO: 21 - protein, 9 aa, Artificial Sequence
  DLL3#4 LCCDR3
QHSRELPWT

SEQ ID NO: 22 - protein, 10 aa, Artificial Sequence
  DLL3#4 HCCDR1
VYTFTSYFMY

SEQ ID NO: 23 - protein, 17 aa, Artificial Sequence
  DLL3#4 HCCDR2
EISPTNGNSNLNERFKN

SEQ ID NO: 24 - protein, 8 aa, Artificial Sequence
  DLL3#4 HCCDR3
GGDGYLDY

SEQ ID NO: 25 - protein, 11 aa, Artificial Sequence
  DLL3#5 LCCDR1
QASQDISNYLN

SEQ ID NO: 26 - protein, 7 aa, Artificial Sequence
  DLL3#5 LCCDR2
DASNLET

SEQ ID NO: 27 - protein, 10 aa, Artificial Sequence
  DLL3#5 LCCDR3
QQYDNLPTWT

SEQ ID NO: 28 - protein, 10 aa, Artificial Sequence
  DLL3#5 HCCDR1
GFTFTGYYIH

SEQ ID NO: 29 - protein, 17 aa, Artificial Sequence
  DLL3#5 HCCDR2
WINPNSGGTNYAQKFQG

SEQ ID NO: 30 - protein, 4 aa, Artificial Sequence
  DLL3#5 HCCDR3
GWDY

SEQ ID NO: 31 - protein, 11 aa, Artificial Sequence
  DLL3#6 LCCDR1
RASQDISNYFA

SEQ ID NO: 32 - protein, 7 aa, Artificial Sequence
  DLL3#6 LCCDR2
AASTLQS

SEQ ID NO: 33 - protein, 9 aa, Artificial Sequence
  DLL3#6 LCCDR3
QQLNSYPYT

SEQ ID NO: 34 - protein, 10 aa, Artificial Sequence
  DLL3#6 HCCDR1
GGSISSYFWS

SEQ ID NO: 35 - protein, 16 aa, Artificial Sequence
  DLL3#6 HCCDR2
RIYTSGSTNYNPSLNS

SEQ ID NO: 36 - protein, 9 aa, Artificial Sequence
  DLL3#6 HCCDR3
RGDWGGFDI

SEQ ID NO: 37 - protein, 108 aa, Artificial Sequence
  DLL3#1 VL
EIVLTQSPGTLSLSPGERATLSCRASQSVSSNFLVWYQQKPGQAPRPLIYGASTRASGIPDRFSGSGSGADFTLTISRLEPEDFALYYCQQYGDSPYTFGQGTTLEIK

SEQ ID NO: 38 - protein, 121 aa, Artificial Sequence
  DLL3#1 VH
QVQLVQSGAEVKKPGASVKVSCKASGNTFTNYYMHWVRQAPGPGLEWMGIIDPSVGSKSYAQKFLGRVTIARDTSTSTVFLDLYSLRSEDTAVYFCARAGKRFGESYFDYWGQGTLVTVSS

SEQ ID NO: 39 - protein, 107 aa, Artificial Sequence
  DLL3#2 VL
DIQMTQSPSAMSASVGDRVTITCRASQGISNYLAWFQQKPGKVPEPLIYAASSLQSGVPSRFSGSGSVTEFTLTISSLQPEDFATYYCLQHNSSPYTFGQGTKLEIK

SEQ ID NO: 40 - protein, 124 aa, Artificial Sequence
  DLL3#2 VH
QVQLVQSGAEVKKPGASVKVSCKASGYTFTSYYMHWVRQAPGQGLEWMGIINPSGGSTSYAQKFQGRVTMTRDTSTSTVYMELSSLRSEDTAVYYCARGEAVGGNYYYYGMDVWGQGTTVTVSS

SEQ ID NO: 41 - protein, 107 aa, Artificial Sequence
  DLL3#3 VL
DIQMTQSPSAMSASVGDRVTITCRASQGISNYLVWFQQKPGKAPKRLIYAVSSLYSGVPSRFSGSGSGTEFTLTISSLQPEDFATYYCLQHDSYPYTFGQGTKLEIK

SEQ ID NO: 42 - protein, 124 aa, Artificial Sequence
  DLL3#3 VH
QVQLVQSGAEVKKPGASVKVSCKASGYTFTSYYVHWVRQAPGQGLEWMVIINPGGGTTSYAQKFLGRVTMTRDTSTNTVYMELKSLRSEDTAVYYCARGEAVTGNYFYYGMDVWGQGTTVTVSS

SEQ ID NO: 43 - protein, 111 aa, Artificial Sequence
  DLL3#4 VL
DIVLTQSPASLAVSLGQRATISCRASKSVSSFGYSFMHWYQQKPGQPPKLLIYLASNLESGVPARFSGSGSGTDFTLNIHPVEEEDAATYYCQHSRELPWTFGGGTKLEIK

SEQ ID NO: 44 - protein, 117 aa, Artificial Sequence
  DLL3#4 VH
QVQLQQSGTELVKPGASVKLSCKASVYTFTSYFMYWVKQRPGHGLEWIGEISPTNGNSNLNERFKNKATLTVDKSSSTAYMQLSSLTSEDSAVYYCTRGGDGYLDYWGQGTTLTVSS

SEQ ID NO: 45 - protein, 108 aa, Artificial Sequence
  DLL3#5 VL
DIQMTQSPSSLSASVGDRVTVTCQASQDISNYLNWYQQKPGKAPKLLIYDASNLETGVPSRFSGSGSGTDFTFTISSLQPEDIATYYCQQYDNLPTWTFGQGTKVEIK

SEQ ID NO: 46 - protein, 113 aa, Artificial Sequence
  DLL3#5 VH
QVQLVQSGAEVKKPGASVKVSCKASGFTFTGYYIHWVRQAPGQGLEWMGWINPNSGGTNYAQKFQGRVTMTRDSSINTAFMELSRLTSDDTAVYYCAAGWDYWGQGTLVTVSS

SEQ ID NO: 47 - protein, 107 aa, Artificial Sequence
  DLL3#6 VL
DIQLTQSPSFLSTSVGDRVTITCRASQDISNYFAWYQQKPGKAPKLLIYAASTLQSGVPSRFSGGGSGTEFTLTISSLQPEDFATYYCQQLNSYPYTFGQGTKLEIK

SEQ ID NO: 48 - protein, 117 aa, Artificial Sequence
  DLL3#6 VH
QVQLQESGPGLVKPSETLSLTCTVSGGSISSYFWSWIRQPAGKGLEWIGRIYTSGSTNYNPSLNSRLTMSVDTSKNQFSLKLSSVTAADTAVYYCARRGDWGGFDIWGQGTVVTVSS

SEQ ID NO: 49 - protein, 477 aa, Artificial Sequence
  DLL3#1 scFab
EIVLTQSPGTLSLSPGERATLSCRASQSVSSNFLVWYQQKPGQAPRPLIYGASTRASGIPDRFSGSGSGADFTLTISRLEPEDFALYYCQQYGDSPYTFGQGTTLEIKRTVAAPSVFIFPPSDEQLKSGTASVVCLLNNFYPREAKVQWKVDNALQSGNSQESVTEQDSKDSTYSLSSTLTLSKADYEKHKVYACEVTHQGLSSPVTKSFNRGECGGGGSEGKSSGSGSESKSTEGKSSGSGSESKSTGGGGSQVQLVQSGAEVKKPGASVKVSCKASGNTFTNYYMHWVRQAPGPGLEWMGIIDPSVGSKSYAQKFLGRVTIARDTSTSTVFLDLYSLRSEDTAVYFCARAGKRFGESYFDYWGQGTLVTVSSASTKGPSVFPLAPSSKSTSGGTAALGCLVKDYFPEPVTVSWNSGALTSGVHTFPAVLQSSGLYSLSSVVTVPSSSLGTQTYICNVNHKPSNTKVDKRVEPKSC

SEQ ID NO: 50 - protein, 479 aa, Artificial Sequence
  DLL3#2 scFab
DIQMTQSPSAMSASVGDRVTITCRASQGISNYLAWFQQKPGKVPEPLIYAASSLQSGVPSRFSGSGSVTEFTLTISSLQPEDFATYYCLQHNSSPYTFGQGTKLEIKRTVAAPSVFIFPPSDEQLKSGTASVVCLLNNFYPREAKVQWKVDNALQSGNSQESVTEQDSKDSTYSLSSTLTLSKADYEKHKVYACEVTHQGLSSPVTKSFNRGECGGGGSEGKSSGSGSESKSTEGKSSGSGSESKSTGGGGSQVQLVQSGAEVKKPGASVKVSCKASGYTFTSYYMHWVRQAPGQGLEWMGIINPSGGSTSYAQKFQGRVTMTRDTSTSTVYMELSSLRSEDTAVYYCARGEAVGGNYYYYGMDVWGQGTTVTVSSASTKGPSVFPLAPSSKSTSGGTAALGCLVKDYFPEPVTVSWNSGALTSGVHTFPAVLQSSGLYSLSSVVTVPSSSLGTQTYICNVNHKPSNTKVDKRVEPKSC

SEQ ID NO: 51 - protein, 479 aa, Artificial Sequence
  DLL3#3 scFab
DIQMTQSPSAMSASVGDRVTITCRASQGISNYLVWFQQKPGKAPKRLIYAVSSLYSGVPSRFSGSGSGTEFTLTISSLQPEDFATYYCLQHDSYPYTFGQGTKLEIKRTVAAPSVFIFPPSDEQLKSGTASVVCLLNNFYPREAKVQWKVDNALQSGNSQESVTEQDSKDSTYSLSSTLTLSKADYEKHKVYACEVTHQGLSSPVTKSFNRGECGGGGSEGKSSGSGSESKSTEGKSSGSGSESKSTGGGGSQVQLVQSGAEVKKPGASVKVSCKASGYTFTSYYVHWVRQAPGQGLEWMVIINPGGGTTSYAQKFLGRVTMTRDTSTNTVYMELKSLRSEDTAVYYCARGEAVTGNYFYYGMDVWGQGTTVTVSSASTKGPSVFPLAPSSKSTSGGTAALGCLVKDYFPEPVTVSWNSGALTSGVHTFPAVLQSSGLYSLSSVVTVPSSSLGTQTYICNVNHKPSNTKVDKRVEPKSC

SEQ ID NO: 52 - protein, 476 aa, Artificial Sequence
  DLL3#4 scFab
DIVLTQSPASLAVSLGQRATISCRASKSVSSFGYSFMHWYQQKPGQPPKLLIYLASNLESGVPARFSGSGSGTDFTLNIHPVEEEDAATYYCQHSRELPWTFGGGTKLEIKRTVAAPSVFIFPPSDEQLKSGTASVVCLLNNFYPREAKVQWKVDNALQSGNSQESVTEQDSKDSTYSLSSTLTLSKADYEKHKVYACEVTHQGLSSPVTKSFNRGECGGGGSEGKSSGSGSESKSTEGKSSGSGSESKSTGGGGSQVQLQQSGTELVKPGASVKLSCKASVYTFTSYFMYWVKQRPGHGLEWIGEISPTNGNSNLNERFKNKATLTVDKSSSTAYMQLSSLTSEDSAVYYCTRGGDGYLDYWGQGTTLTVSSASTKGPSVFPLAPSSKSTSGGTAALGCLVKDYFPEPVTVSWNSGALTSGVHTFPAVLQSSGLYSLSSVVTVPSSSLGTQTYICNVNHKPSNTKVDKRVEPKSC

SEQ ID NO: 53 - protein, 469 aa, Artificial Sequence
  DLL3#5 scFab
DIQMTQSPSSLSASVGDRVTVTCQASQDISNYLNWYQQKPGKAPKLLIYDASNLETGVPSRFSGSGSGTDFTFTISSLQPEDIATYYCQQYDNLPTWTFGQGTKVEIKRTVAAPSVFIFPPSDEQLKSGTASVVCLLNNFYPREAKVQWKVDNALQSGNSQESVTEQDSKDSTYSLSSTLTLSKADYEKHKVYACEVTHQGLSSPVTKSFNRGECGGGGSEGKSSGSGSESKSTEGKSSGSGSESKSTGGGGSQVQLVQSGAEVKKPGASVKVSCKASGFTFTGYYIHWVRQAPGQGLEWMGWINPNSGGTNYAQKFQGRVTMTRDSSINTAFMELSRLTSDDTAVYYCAAGWDYWGQGTLVTVSSASTKGPSVFPLAPSSKSTSGGTAALGCLVKDYFPEPVTVSWNSGALTSGVHTFPAVLQSSGLYSLSSVVTVPSSSLGTQTYICNVNHKPSNTKVDKRVEPKSC

SEQ ID NO: 54 - protein, 472 aa, Artificial Sequence
  DLL3#6 scFab
DIQLTQSPSFLSTSVGDRVTITCRASQDISNYFAWYQQKPGKAPKLLIYAASTLQSGVPSRFSGGGSGTEFTLTISSLQPEDFATYYCQQLNSYPYTFGQGTKLEIKRTVAAPSVFIFPPSDEQLKSGTASVVCLLNNFYPREAKVQWKVDNALQSGNSQESVTEQDSKDSTYSLSSTLTLSKADYEKHKVYACEVTHQGLSSPVTKSFNRGECGGGGSEGKSSGSGSESKSTEGKSSGSGSESKSTGGGGSQVQLQESGPGLVKPSETLSLTCTVSGGSISSYFWSWIRQPAGKGLEWIGRIYTSGSTNYNPSLNSRLTMSVDTSKNQFSLKLSSVTAADTAVYYCARRGDWGGFDIWGQGTVVTVSSASTKGPSVFPLAPSSKSTSGGTAALGCLVKDYFPEPVTVSWNSGALTSGVHTFPAVLQSSGLYSLSSVVTVPSSSLGTQTYICNVNHKPSNTKVDKRVEPKSC

SEQ ID NO: 55 - protein, 14 aa, Artificial Sequence
  CD3#1 LCCDR1
RSSTGAVTTSNYAN

SEQ ID NO: 56 - protein, 7 aa, Artificial Sequence
  CD3#1 LCCDR2
GTNKRAP

SEQ ID NO: 57 - protein, 9 aa, Artificial Sequence
  CD3#1 LCCDR3
ALWYSNLWV

SEQ ID NO: 58 - protein, 10 aa, Artificial Sequence
  CD3#1 HCCDR1
GFTFNTYAMN

SEQ ID NO: 59 - protein, 19 aa, Artificial Sequence
  CD3#1 HCCDR2
RIRSKYNNYATYYADSVKD

SEQ ID NO: 60 - protein, 14 aa, Artificial Sequence
  CD3#1 HCCDR3
HGNFGNSYVSWFAY

SEQ ID NO: 61 - protein, 14 aa, Artificial Sequence
  CD3#2 LCCDR1
RSSTGAVTTSNYAN

SEQ ID NO: 62 - protein, 7 aa, Artificial Sequence
  CD3#2 LCCDR2
GTNKRAP

SEQ ID NO: 63 - protein, 9 aa, Artificial Sequence
  CD3#2 LCCDR3
ALWYSNLWV

SEQ ID NO: 64 - protein, 10 aa, Artificial Sequence
  CD3#2 HCCDR1
GFTFNTYAMN

SEQ ID NO: 65 - protein, 19 aa, Artificial Sequence
  CD3#2 HCCDR2
RIRSKYINYATYYADSVKD

SEQ ID NO: 66 - protein, 14 aa, Artificial Sequence
  CD3#2 HCCDR3
HGNFGNSYVSWFAY

SEQ ID NO: 67 - protein, 109 aa, Artificial Sequence
  CD3#1 VL
EAVVTQEPSLTVSPGGTVTLTCRSSTGAVTTSNYANWVQEKPGQLPRGLIGGTNKRAPWVPARFSGSLLGGKAALTLSGAQPEDEAEYFCALWYSNLWVFGGGTKLTVL

SEQ ID NO: 68 - protein, 125 aa, Artificial Sequence
  CD3#1 VH
EVQLVESGGGLVQPGGSLKLSCAASGFTFNTYAMNWVRQAPGKGLEWVARIRSKYNNYATYYADSVKDRFTISRDDSKNTAYLQMNNLKTEDTAVYYCVRHGNFGNSYVSWFAYWGQGTLVTVSA

SEQ ID NO: 69 - protein, 109 aa, Artificial Sequence; identical to SEQ ID NO: 67
  CD3#2 VL

SEQ ID NO: 70 - protein, 125 aa, Artificial Sequence
  CD3#2 VH
EVQLVESGGGLVQPGGSLKLSCAASGFTFNTYAMNWVRQAPGKGLEWVARIRSKYINYATYYADSVKDRFTISRDDSKNTAYLQMNNLKTEDTAVYYCVRHGNFGNSYVSWFAYWGQGTLVTVSA

SEQ ID NO: 71 - protein, 481 aa, Artificial Sequence
  CD3#1 scFab
EAVVTQEPSLTVSPGGTVTLTCRSSTGAVTTSNYANWVQEKPGQLPRGLIGGTNKRAPWVPARFSGSLLGGKAALTLSGAQPEDEAEYFCALWYSNLWVFGGGTKLTVLGQPKAAPSVTLFPPSSEELQANKATLVCLISDFYPGAVKVAWKADGSPVNTGVETTTPSKQSNNKYAASSYLSLTPEQWKSHRSYSCQVTHEGSTVEKTVAPAECSGGGGSEGKSSGSGSESKSTEGKSSGSGSESKSTGGGGSEVQLVESGGGLVQPGGSLKLSCAASGFTFNTYAMNWVRQAPGKGLEWVARIRSKYNNYATYYADSVKDRFTISRDDSKNTAYLQMNNLKTEDTAVYYCVRHGNFGNSYVSWFAYWGQGTLVTVSAASTKGPSVFPLAPSSKSTSGGTAALGCLVKDYFPEPVTVSWNSGALTSGVHTFPAVLQSSGLYSLSSVVTVPSSSLGTQTYICNVNHKPSNTKVDKRVEPKSC

SEQ ID NO: 72 - protein, 481 aa, Artificial Sequence
  CD3#2 scFab
EAVVTQEPSLTVSPGGTVTLTCRSSTGAVTTSNYANWVQEKPGQLPRGLIGGTNKRAPWVPARFSGSLLGGKAALTLSGAQPEDEAEYFCALWYSNLWVFGGGTKLTVLGQPKAAPSVTLFPPSSEELQANKATLVCLISDFYPGAVKVAWKADGSPVNTGVETTTPSKQSNNKYAASSYLSLTPEQWKSHRSYSCQVTHEGSTVEKTVAPAECSGGGGSEGKSSGSGSESKSTEGKSSGSGSESKSTGGGGSEVQLVESGGGLVQPGGSLKLSCAASGFTFNTYAMNWVRQAPGKGLEWVARIRSKYINYATYYADSVKDRFTISRDDSKNTAYLQMNNLKTEDTAVYYCVRHGNFGNSYVSWFAYWGQGTLVTVSAASTKGPSVFPLAPSSKSTSGGTAALGCLVKDYFPEPVTVSWNSGALTSGVHTFPAVLQSSGLYSLSSVVTVPSSSLGTQTYICNVNHKPSNTKVDKRVEPKSC

SEQ ID NO: 73 - protein, 703 aa, Artificial Sequence
  DLL3#1 chain
EIVLTQSPGTLSLSPGERATLSCRASQSVSSNFLVWYQQKPGQAPRPLIYGASTRASGIPDRFSGSGSGADFTLTISRLEPEDFALYYCQQYGDSPYTFGQGTTLEIKRTVAAPSVFIFPPSDEQLKSGTASVVCLLNNFYPREAKVQWKVDNALQSGNSQESVTEQDSKDSTYSLSSTLTLSKADYEKHKVYACEVTHQGLSSPVTKSFNRGECGGGGSEGKSSGSGSESKSTEGKSSGSGSESKSTGGGGSQVQLVQSGAEVKKPGASVKVSCKASGNTFTNYYMHWVRQAPGPGLEWMGIIDPSVGSKSYAQKFLGRVTIARDTSTSTVFLDLYSLRSEDTAVYFCARAGKRFGESYFDYWGQGTLVTVSSASTKGPSVFPLAPSSKSTSGGTAALGCLVKDYFPEPVTVSWNSGALTSGVHTFPAVLQSSGLYSLSSVVTVPSSSLGTQTYICNVNHKPSNTKVDKRVEPKSCDKTHTCPPCPAPEAAGGPSVFLFPPKPKDTLMISRTPEVTCVVVDVSHEDPEVKFNWYVDGVEVHNAKTKPREEQYNSTYRVVSVLTVLHQDWLNGKEYKCKVSNKALPAPIEKTISKAKGQPREPQVYTLPPSREEMTKNQVSLWCLVKGFYPSDIAVEWESNGQPENNYKTTPPVLDSDGSFFLYSKLTVDKSRWQQGNVFSCSVMHEALHNHYTQKSLSLSPG

SEQ ID NO: 74 - protein, 705 aa, Artificial Sequence
  DLL3#2 chain
DIQMTQSPSAMSASVGDRVTITCRASQGISNYLAWFQQKPGKVPEPLIYAASSLQSGVPSRFSGSGSVTEFTLTISSLQPEDFATYYCLQHNSSPYTFGQGTKLEIKRTVAAPSVFIFPPSDEQLKSGTASVVCLLNNFYPREAKVQWKVDNALQSGNSQESVTEQDSKDSTYSLSSTLTLSKADYEKHKVYACEVTHQGLSSPVTKSFNRGECGGGGSEGKSSGSGSESKSTEGKSSGSGSESKSTGGGGSQVQLVQSGAEVKKPGASVKVSCKASGYTFTSYYMHWVRQAPGQGLEWMGIINPSGGSTSYAQKFQGRVTMTRDTSTSTVYMELSSLRSEDTAVYYCARGEAVGGNYYYYGMDVWGQGTTVTVSSASTKGPSVFPLAPSSKSTSGGTAALGCLVKDYFPEPVTVSWNSGALTSGVHTFPAVLQSSGLYSLSSVVTVPSSSLGTQTYICNVNHKPSNTKVDKRVEPKSCDKTHTCPPCPAPEAAGGPSVFLFPPKPKDTLMISRTPEVTCVVVDVSHEDPEVKFNWYVDGVEVHNAKTKPREEQYNSTYRVVSVLTVLHQDWLNGKEYKCKVSNKALPAPIEKTISKAKGQPREPQVYTLPPSREEMTKNQVSLWCLVKGFYPSDIAVEWESNGQPENNYKTTPPVLDSDGSFFLYSKLTVDKSRWQQGNVFSCSVMHEALHNHYTQKSLSLSPG

SEQ ID NO: 75 - protein, 705 aa, Artificial Sequence
  DLL3#3 chain
DIQMTQSPSAMSASVGDRVTITCRASQGISNYLVWFQQKPGKAPKRLIYAVSSLYSGVPSRFSGSGSGTEFTLTISSLQPEDFATYYCLQHDSYPYTFGQGTKLEIKRTVAAPSVFIFPPSDEQLKSGTASVVCLLNNFYPREAKVQWKVDNALQSGNSQESVTEQDSKDSTYSLSSTLTLSKADYEKHKVYACEVTHQGLSSPVTKSFNRGECGGGGSEGKSSGSGSESKSTEGKSSGSGSESKSTGGGGSQVQLVQSGAEVKKPGASVKVSCKASGYTFTSYYVHWVRQAPGQGLEWMVIINPGGGTTSYAQKFLGRVTMTRDTSTNTVYMELKSLRSEDTAVYYCARGEAVTGNYFYYGMDVWGQGTTVTVSSASTKGPSVFPLAPSSKSTSGGTAALGCLVKDYFPEPVTVSWNSGALTSGVHTFPAVLQSSGLYSLSSVVTVPSSSLGTQTYICNVNHKPSNTKVDKRVEPKSCDKTHTCPPCPAPEAAGGPSVFLFPPKPKDTLMISRTPEVTCVVVDVSHEDPEVKFNWYVDGVEVHNAKTKPREEQYNSTYRVVSVLTVLHQDWLNGKEYKCKVSNKALPAPIEKTISKAKGQPREPQVYTLPPSREEMTKNQVSLWCLVKGFYPSDIAVEWESNGQPENNYKTTPPVLDSDGSFFLYSKLTVDKSRWQQGNVFSCSVMHEALHNHYTQKSLSLSPG

SEQ ID NO: 76 - protein, 702 aa, Artificial Sequence
  DLL3#4 chain
DIVLTQSPASLAVSLGQRATISCRASKSVSSFGYSFMHWYQQKPGQPPKLLIYLASNLESGVPARFSGSGSGTDFTLNIHPVEEEDAATYYCQHSRELPWTFGGGTKLEIKRTVAAPSVFIFPPSDEQLKSGTASVVCLLNNFYPREAKVQWKVDNALQSGNSQESVTEQDSKDSTYSLSSTLTLSKADYEKHKVYACEVTHQGLSSPVTKSFNRGECGGGGSEGKSSGSGSESKSTEGKSSGSGSESKSTGGGGSQVQLQQSGTELVKPGASVKLSCKASVYTFTSYFMYWVKQRPGHGLEWIGEISPTNGNSNLNERFKNKATLTVDKSSSTAYMQLSSLTSEDSAVYYCTRGGDGYLDYWGQGTTLTVSSASTKGPSVFPLAPSSKSTSGGTAALGCLVKDYFPEPVTVSWNSGALTSGVHTFPAVLQSSGLYSLSSVVTVPSSSLGTQTYICNVNHKPSNTKVDKRVEPKSCDKTHTCPPCPAPEAAGGPSVFLFPPKPKDTLMISRTPEVTCVVVDVSHEDPEVKFNWYVDGVEVHNAKTKPREEQYNSTYRVVSVLTVLHQDWLNGKEYKCKVSNKALPAPIEKTISKAKGQPREPQVYTLPPSREEMTKNQVSLWCLVKGFYPSDIAVEWESNGQPENNYKTTPPVLDSDGSFFLYSKLTVDKSRWQQGNVFSCSVMHEALHNHYTQKSLSLSPG

SEQ ID NO: 77 - protein, 695 aa, Artificial Sequence
  DLL3#5 chain
DIQMTQSPSSLSASVGDRVTVTCQASQDISNYLNWYQQKPGKAPKLLIYDASNLETGVPSRFSGSGSGTDFTFTISSLQPEDIATYYCQQYDNLPTWTFGQGTKVEIKRTVAAPSVFIFPPSDEQLKSGTASVVCLLNNFYPREAKVQWKVDNALQSGNSQESVTEQDSKDSTYSLSSTLTLSKADYEKHKVYACEVTHQGLSSPVTKSFNRGECGGGGSEGKSSGSGSESKSTEGKSSGSGSESKSTGGGGSQVQLVQSGAEVKKPGASVKVSCKASGFTFTGYYIHWVRQAPGQGLEWMGWINPNSGGTNYAQKFQGRVTMTRDSSINTAFMELSRLTSDDTAVYYCAAGWDYWGQGTLVTVSSASTKGPSVFPLAPSSKSTSGGTAALGCLVKDYFPEPVTVSWNSGALTSGVHTFPAVLQSSGLYSLSSVVTVPSSSLGTQTYICNVNHKPSNTKVDKRVEPKSCDKTHTCPPCPAPEAAGGPSVFLFPPKPKDTLMISRTPEVTCVVVDVSHEDPEVKFNWYVDGVEVHNAKTKPREEQYNSTYRVVSVLTVLHQDWLNGKEYKCKVSNKALPAPIEKTISKAKGQPREPQVYTLPPSREEMTKNQVSLWCLVKGFYPSDIAVEWESNGQPENNYKTTPPVLDSDGSFFLYSKLTVDKSRWQQGNVFSCSVMHEALHNHYTQKSLSLSPG

SEQ ID NO: 78 - protein, 698 aa, Artificial Sequence
  DLL3#6 chain
DIQLTQSPSFLSTSVGDRVTITCRASQDISNYFAWYQQKPGKAPKLLIYAASTLQSGVPSRFSGGGSGTEFTLTISSLQPEDFATYYCQQLNSYPYTFGQGTKLEIKRTVAAPSVFIFPPSDEQLKSGTASVVCLLNNFYPREAKVQWKVDNALQSGNSQESVTEQDSKDSTYSLSSTLTLSKADYEKHKVYACEVTHQGLSSPVTKSFNRGECGGGGSEGKSSGSGSESKSTEGKSSGSGSESKSTGGGGSQVQLQESGPGLVKPSETLSLTCTVSGGSISSYFWSWIRQPAGKGLEWIGRIYTSGSTNYNPSLNSRLTMSVDTSKNQFSLKLSSVTAADTAVYYCARRGDWGGFDIWGQGTVVTVSSASTKGPSVFPLAPSSKSTSGGTAALGCLVKDYFPEPVTVSWNSGALTSGVHTFPAVLQSSGLYSLSSVVTVPSSSLGTQTYICNVNHKPSNTKVDKRVEPKSCDKTHTCPPCPAPEAAGGPSVFLFPPKPKDTLMISRTPEVTCVVVDVSHEDPEVKFNWYVDGVEVHNAKTKPREEQYNSTYRVVSVLTVLHQDWLNGKEYKCKVSNKALPAPIEKTISKAKGQPREPQVYTLPPSREEMTKNQVSLWCLVKGFYPSDIAVEWESNGQPENNYKTTPPVLDSDGSFFLYSKLTVDKSRWQQGNVFSCSVMHEALHNHYTQKSLSLSPG

SEQ ID NO: 79 - protein, 707 aa, Artificial Sequence
  CD3#1 chain
EAVVTQEPSLTVSPGGTVTLTCRSSTGAVTTSNYANWVQEKPGQLPRGLIGGTNKRAPWVPARFSGSLLGGKAALTLSGAQPEDEAEYFCALWYSNLWVFGGGTKLTVLGQPKAAPSVTLFPPSSEELQANKATLVCLISDFYPGAVKVAWKADGSPVNTGVETTTPSKQSNNKYAASSYLSLTPEQWKSHRSYSCQVTHEGSTVEKTVAPAECSGGGGSEGKSSGSGSESKSTEGKSSGSGSESKSTGGGGSEVQLVESGGGLVQPGGSLKLSCAASGFTFNTYAMNWVRQAPGKGLEWVARIRSKYNNYATYYADSVKDRFTISRDDSKNTAYLQMNNLKTEDTAVYYCVRHGNFGNSYVSWFAYWGQGTLVTVSAASTKGPSVFPLAPSSKSTSGGTAALGCLVKDYFPEPVTVSWNSGALTSGVHTFPAVLQSSGLYSLSSVVTVPSSSLGTQTYICNVNHKPSNTKVDKRVEPKSCDKTHTCPPCPAPEAAGGPSVFLFPPKPKDTLMISRTPEVTCVVVDVSHEDPEVKFNWYVDGVEVHNAKTKPREEQYNSTYRVVSVLTVLHQDWLNGKEYKCKVSNKALPAPIEKTISKAKGQPREPQVYTLPPSREEMTKNQVSLSCAVKGFYPSDIAVEWESNGQPENNYKTTPPVLDSDGSFFLVSKLTVDKSRWQQGNVFSCSVMHEALHNRFTQKSLSLSPG

SEQ ID NO: 80 - protein, 707 aa, Artificial Sequence
  CD3#2 chain
EAVVTQEPSLTVSPGGTVTLTCRSSTGAVTTSNYANWVQEKPGQLPRGLIGGTNKRAPWVPARFSGSLLGGKAALTLSGAQPEDEAEYFCALWYSNLWVFGGGTKLTVLGQPKAAPSVTLFPPSSEELQANKATLVCLISDFYPGAVKVAWKADGSPVNTGVETTTPSKQSNNKYAASSYLSLTPEQWKSHRSYSCQVTHEGSTVEKTVAPAECSGGGGSEGKSSGSGSESKSTEGKSSGSGSESKSTGGGGSEVQLVESGGGLVQPGGSLKLSCAASGFTFNTYAMNWVRQAPGKGLEWVARIRSKYINYATYYADSVKDRFTISRDDSKNTAYLQMNNLKTEDTAVYYCVRHGNFGNSYVSWFAYWGQGTLVTVSAASTKGPSVFPLAPSSKSTSGGTAALGCLVKDYFPEPVTVSWNSGALTSGVHTFPAVLQSSGLYSLSSVVTVPSSSLGTQTYICNVNHKPSNTKVDKRVEPKSCDKTHTCPPCPAPEAAGGPSVFLFPPKPKDTLMISRTPEVTCVVVDVSHEDPEVKFNWYVDGVEVHNAKTKPREEQYNSTYRVVSVLTVLHQDWLNGKEYKCKVSNKALPAPIEKTISKAKGQPREPQVYTLPPSREEMTKNQVSLSCAVKGFYPSDIAVEWESNGQPENNYKTTPPVLDSDGSFFLVSKLTVDKSRWQQGNVFSCSVMHEALHNRFTQKSLSLSPG

SEQ ID NO: 81 - protein, 226 aa, Artificial Sequence
  Fcdomain* (IgG1)
DKTHTCPPCPAPELLGGPSVFLFPPKPKDTLMISRTPEVTCVVVDVSHEDPEVKFNWYVDGVEVHNAKTKPREEQYNSTYRVVSVLTVLHQDWLNGKEYKCKVSNKALPAPIEKTISKAKGQPREPQVYTLPPSREEMTKNQVSLTCLVKGFYPSDIAVEWESNGQPENNYKTTPPVLDSDGSFFLYSKLTVDKSRWQQGNVFSCSVMHEALHNHYTQKSLSLSPG

SEQ ID NO: 82 - protein, 226 aa, Artificial Sequence
  Fcknobdomain (IgG1,LALA)
DKTHTCPPCPAPEAAGGPSVFLFPPKPKDTLMISRTPEVTCVVVDVSHEDPEVKFNWYVDGVEVHNAKTKPREEQYNSTYRVVSVLTVLHQDWLNGKEYKCKVSNKALPAPIEKTISKAKGQPREPQVYTLPPSREEMTKNQVSLWCLVKGFYPSDIAVEWESNGQPENNYKTTPPVLDSDGSFFLYSKLTVDKSRWQQGNVFSCSVMHEALHNHYTQKSLSLSPG

SEQ ID NO: 83 - protein, 226 aa, Artificial Sequence
  Fcholedomain (IgG1,RF/LALA)
DKTHTCPPCPAPEAAGGPSVFLFPPKPKDTLMISRTPEVTCVVVDVSHEDPEVKFNWYVDGVEVHNAKTKPREEQYNSTYRVVSVLTVLHQDWLNGKEYKCKVSNKALPAPIEKTISKAKGQPREPQVYTLPPSREEMTKNQVSLSCAVKGFYPSDIAVEWESNGQPENNYKTTPPVLDSDGSFFLVSKLTVDKSRWQQGNVFSCSVMHEALHNRFTQKSLSLSPG

SEQ ID NO: 84 - protein, 228 aa, Artificial Sequence
  Fcdomain (IgG4Pro)
ESKYGPPCPPCPAPEFLGGPSVFLFPPKPKDTLMISRTPEVTCVVVDVSQEDPEVQFNWYVDGVEVHNAKTKPREEQFNSTYRVVSVLTVLHQDWLNGKEYKCKVSNKGLPSSIEKTISKAKGQPREPQVYTLPPSQEEMTKNQVSLTCLVKGFYPSDIAVEWESNGQPENNYKTTPPVLDSDGSFFLYSRLTVDKSRWQEGNVFSCSVMHEALHNHYTQKSLSLSLG

SEQ ID NO: 85 - protein, 228 aa, Artificial Sequence
  Fcknobdomain(IgG4Pro)
ESKYGPPCPPCPAPEFLGGPSVFLFPPKPKDTLMISRTPEVTCVVVDVSQEDPEVQFNWYVDGVEVHNAKTKPREEQFNSTYRVVSVLTVLHQDWLNGKEYKCKVSNKGLPSSIEKTISKAKGQPREPQVYTLPPSQEEMTKNQVSLWCLVKGFYPSDIAVEWESNGQPENNYKTTPPVLDSDGSFFLYSRLTVDKSRWQEGNVFSCSVMHEALHNHYTQKSLSLSLG

SEQ ID NO: 86 - protein, 228 aa, Artificial Sequence
  Fcholedomain(IgG4Pro,RF)
ESKYGPPCPPCPAPEFLGGPSVFLFPPKPKDTLMISRTPEVTCVVVDVSQEDPEVQFNWYVDGVEVHNAKTKPREEQFNSTYRVVSVLTVLHQDWLNGKEYKCKVSNKGLPSSIEKTISKAKGQPREPQVYTLPPSQEEMTKNQVSLSCAVKGFYPSDIAVEWESNGQPENNYKTTPPVLDSDGSFFLVSRLTVDKSRWQEGNVFSCSVMHEALHNRFTQKSLSLSLG

SEQ ID NO: 87 - protein, 107 aa, Artificial Sequence [sequence omitted]

SEQ ID NO: 88 - protein, 106 aa, Artificial Sequence
  constantregionofalambdalightchain
GQPKAAPSVTLFPPSSEELQANKATLVCLISDFYPGAVKVAWKADGSPVNTGVETTTPSKQSNNKYAASSYLSLTPEQWKSHRSYSCQVTHEGSTVEKTVAPAECS

SEQ ID NO: 89 - protein, 38 aa, Artificial Sequence
  Linker
GGGGSEGKSSGSGSESKSTEGKSSGSGSESKSTGGGGS

SEQ ID NO: 90 - protein, 22 aa, Artificial Sequence
  Linker
GGGGSGGGGSGGSGGSGGGGGS

SEQ ID NO: 91 - protein, 26 aa, Artificial Sequence
  Linker
GGGGSGGGGSGGGGSGGGGSGGGGGS

SEQ ID NO: 92 - protein, 30 aa, Artificial Sequence
  Linker
GGGGSGGGGGGSGGGGGGSGGGGSGGGGGS

SEQ ID NO: 93 - protein, 34 aa, Artificial Sequence
  Linker
GGGGSGGGGSGGGSGGGSGGGGSGGGGSGGGGGS

SEQ ID NO: 94 - protein, 38 aa, Artificial Sequence
  Linker
GGGGSGGGGSGGGSGGGSGGGSGGGGSGGGGSGGGGGS

SEQ ID NO: 95 - protein, 42 aa, Artificial Sequence
  Linker
GGGGSGGGGSGGGSGGGSGGGSGGGGSGGGGGSGGGSGGGGS

SEQ ID NO: 96 - protein, 14 aa, Artificial Sequence
  CD3#3 LCCDR1
RSSTGAVTTSNYAN

SEQ ID NO: 97 - protein, 7 aa, Artificial Sequence
  CD3#3 LCCDR2
GTNKRAP

SEQ ID NO: 98 - protein, 9 aa, Artificial Sequence
  CD3#3 LCCDR3
ALWYSNLWV

SEQ ID NO: 99 - protein, 10 aa, Artificial Sequence
  CD3#3 HCCDR1
GFTFNTYAMN

SEQ ID NO: 100 - protein, 19 aa, Artificial Sequence
  CD3#3 HCCDR2
RIRSKYANYATYYADSVKD

SEQ ID NO: 101 - protein, 14 aa, Artificial Sequence
  CD3#3 HCCDR3
HGNFGNSYVSWFAY

SEQ ID NO: 102 - protein, 109 aa, Artificial Sequence; identical to SEQ ID NO: 67
  CD3#3 VL

SEQ ID NO: 103 - protein, 125 aa, Artificial Sequence
  CD3#3 HL
EVQLVESGGGLVQPGGSLKLSCAASGFTFNTYAMNWVRQAPGKGLEWVARIRSKYANYATYYADSVKDRFTISRDDSKNTAYLQMNNLKTEDTAVYYCVRHGNFGNSYVSWFAYWGQGTLVTVSA

SEQ ID NO: 104 - protein, 481 aa, Artificial Sequence
  CD3#3 scFab
EAVVTQEPSLTVSPGGTVTLTCRSSTGAVTTSNYANWVQEKPGQLPRGLIGGTNKRAPWVPARFSGSLLGGKAALTLSGAQPEDEAEYFCALWYSNLWVFGGGTKLTVLGQPKAAPSVTLFPPSSEELQANKATLVCLISDFYPGAVKVAWKADGSPVNTGVETTTPSKQSNNKYAASSYLSLTPEQWKSHRSYSCQVTHEGSTVEKTVAPAECSGGGGSEGKSSGSGSESKSTEGKSSGSGSESKSTGGGGSEVQLVESGGGLVQPGGSLKLSCAASGFTFNTYAMNWVRQAPGKGLEWVARIRSKYANYATYYADSVKDRFTISRDDSKNTAYLQMNNLKTEDTAVYYCVRHGNFGNSYVSWFAYWGQGTLVTVSAASTKGPSVFPLAPSSKSTSGGTAALGCLVKDYFPEPVTVSWNSGALTSGVHTFPAVLQSSGLYSLSSVVTVPSSSLGTQTYICNVNHKPSNTKVDKRVEPKSC

SEQ ID NO: 105 - protein, 707 aa, Artificial Sequence
  CD3#3 chain
EAVVTQEPSLTVSPGGTVTLTCRSSTGAVTTSNYANWVQEKPGQLPRGLIGGTNKRAPWVPARFSGSLLGGKAALTLSGAQPEDEAEYFCALWYSNLWVFGGGTKLTVLGQPKAAPSVTLFPPSSEELQANKATLVCLISDFYPGAVKVAWKADGSPVNTGVETTTPSKQSNNKYAASSYLSLTPEQWKSHRSYSCQVTHEGSTVEKTVAPAECSGGGGSEGKSSGSGSESKSTEGKSSGSGSESKSTGGGGSEVQLVESGGGLVQPGGSLKLSCAASGFTFNTYAMNWVRQAPGKGLEWVARIRSKYANYATYYADSVKDRFTISRDDSKNTAYLQMNNLKTEDTAVYYCVRHGNFGNSYVSWFAYWGQGTLVTVSAASTKGPSVFPLAPSSKSTSGGTAALGCLVKDYFPEPVTVSWNSGALTSGVHTFPAVLQSSGLYSLSSVVTVPSSSLGTQTYICNVNHKPSNTKVDKRVEPKSCDKTHTCPPCPAPEAAGGPSVFLFPPKPKDTLMISRTPEVTCVVVDVSHEDPEVKFNWYVDGVEVHNAKTKPREEQYNSTYRVVSVLTVLHQDWLNGKEYKCKVSNKALPAPIEKTISKAKGQPREPQVYTLPPSREEMTKNQVSLSCAVKGFYPSDIAVEWESNGQPENNYKTTPPVLDSDGSFFLVSKLTVDKSRWQQGNVFSCSVMHEALHNRFTQKSLSLSPG

SEQ ID NO: 106 - protein, 476 aa, Artificial Sequence
  HuDLL3(ECD)-His
AGVFELQIHSFGPGPGPGAPRSPCSARLPCRLFFRVCLKPGLSEEAAESPCALGAALSARGPVYTEQPGAPAPDLPLPDGLLQVPFRDAWPGTFSFIIETWREELGDQIGGPAWSLLARVAGRRRLAAGGPWARDIQRAGAWELRFSYRARCEPPAVGTACTRLCRPRSAPSRCGPGLRPCAPLEDECEAPLVCRAGCSPEHGFCEQPGECRCLEGWTGPLCTVPVSTSSCLSPRGPSSATTGCLVPGPGPCDGNPCANGGSCSETPRSFECTCPRGFYGLRCEVSGVTCADGPCFNGGLCVGGADPDSAYICHCPPGFQGSNCEKRVDRCSLQPCRNGGLCLDLGHALRCRCRAGFAGPRCEHDLDDCAGRACANGGTCVEGGGAHRCSCALGFGGRDCRERADPCAARPCAHGGRCYAHFSGLVCACAPGYMGARCEFPVHPDGASALPAAPPGLRPGDPQRYLAGSAHHHHHH

SEQ ID NO: 107 - protein, 476 aa, Artificial Sequence
  CynoDLL3(ECD)-His
AGVFELQIHSFGPGPGPGAPRSPCSARGPCRLFFRVCLKPGLSEEAAESPCALGAALSARGPVYTEQPEAPAPDLPLPNGLLQVPFRDAWPGTFSLIIETWREELGDQIGGPAWSLLARVTRRRRLAAGGPWARDIQRAGAWELRFSYRARCELPAVGTACTRLCRPRSAPSRCGPGLRPCAPLEDECEAPPVCRAGCSLEHGFCEQPGECRCLEGWTGPLCMVPVSTSSCLGLRGPSSTTTGCLVPGPGPCDGNPCANGGSCSETPGSFECTCPRGFYGLRCEVSGVTCADGPCFNGGLCVGGADPDSAYICHCPPGFQGSNCEKRVDRCSLQPCRNGGLCLDLGHALRCRCRAGFAGPRCEHDLDDCAGRACANGGTCVEGGGAHRCSCALGFGGRNCRERADPCAARPCAHGGRCYAHFSGLVCACAPGYMGARCEFPVHPDGVSALPAAPPGLRPGDPQRYLAGSAHHHHHH

SEQ ID NO: 108 - protein, 487 aa, Artificial Sequence
  HuCD3E+G-HuFc-His
QDGNEEMGGITQTPYKVSISGTTVILTCPQYPGSEILWQHNDKNIGGDEDDKNIGSDEDHLSLKEFSELEQSGYYVCYPRGSKPEDANFYLYLRARVCENCMEMDGGGSGGGSGGGSGGGSGGGSGGGSGGQSIKGNHLVKVYDYQEDGSVLLTCDAEAKNITWFKDGKMIGFLTEDKKKWNLGSNAKDPRGMYQCKGSQNKSKPLQVYYRMCQNCIELNAATISGGSGGSGGSGGSGGSGGSGGEPKSCDKTHTCPPCPAPELLGGPSVFLFPPKPKDTLMISRTPEVTCVVVDVSHEDPEVKFNWYVDGVEVHNAKTKPREEQYNSTYRVVSVLTVLHQDWLNGKEYKCKVSNKALPAPIEKTISKAKGQPREPQVYTLPPSRDELTKNQVSLTCLVKGFYPSDIAVEWESNGQPENNYKTTPPVLDSDGSFFLYSKLTVDKSRWQQGNVFSCSVMHEALHNHYTQKSLSLSPGKAGSAHHHHHH

SEQ ID NO: 109 - protein, 477 aa, Artificial Sequence
  CynoCD3E+G-Fc-His
QDGNEEMGSITQTPYQVSISGTTVILTCSQHLGSEAQWQHNGKNKGDSGDQLFLPEFSEMEQSGYYVCYPRGSNPEDASHHLYLKARVCENCMEMDVMGGGSGGGSGGGSGGGSGGGSGGGSGGQSFEENRKLNVYNQEDGSVLLTCHVKNTNITWFKEGKMIDILTAHKNKWNLGSNTKDPRGVYQCKGSKDKSKTLQVYYRMCQNCIELNAATGGSGGSGGSGGSGGSGGSGGEPKSCDKTHTCPPCPAPELLGGPSVFLFPPKPKDTLMISRTPEVTCVVVDVSHEDPEVKFNWYVDGVEVHNAKTKPREEQYNSTYRVVSVLTVLHQDWLNGKEYKCKVSNKALPAPIEKTISKAKGQPREPQVYTLPPSRDELTKNQVSLTCLVKGFYPSDIAVEWESNGQPENNYKTTPPVLDSDGSFFLYSKLTVDKSRWQQGNVFSCSVMHEALHNHYTQKSLSLSPGKAGSAHHHHHH

SEQ ID NO: 110 - protein, 626 aa, Artificial Sequence
  FLAG-tagged human DLL3 full length
MVSPRMSGLLSQTVILALIFLPQTRPDYKDDDDKAGVFELQIHSFGPGPGPGAPRSPCSARLPCRLFFRVCLKPGLSEEAAESPCALGAALSARGPVYTEQPGAPAPDLPLPDGLLQVPFRDAWPGTFSFIIETWREELGDQIGGPAWSLLARVAGRRRLAAGGPWARDIQRAGAWELRFSYRARCEPPAVGTACTRLCRPRSAPSRCGPGLRPCAPLEDECEAPLVCRAGCSPEHGFCEQPGECRCLEGWTGPLCTVPVSTSSCLSPRGPSSATTGCLVPGPGPCDGNPCANGGSCSETPRSFECTCPRGFYGLRCEVSGVTCADGPCFNGGLCVGGADPDSAYICHCPPGFQGSNCEKRVDRCSLQPCRNGGLCLDLGHALRCRCRAGFAGPRCEHDLDDCAGRACANGGTCVEGGGAHRCSCALGFGGRDCRERADPCAARPCAHGGRCYAHFSGLVCACAPGYMGARCEFPVHPDGASALPAAPPGLRPGDPQRYLLPPALGLLVAAGVAGAALLLVHVRRRGHSQDAGSRLLAGTPEPSVHALPDALNNLRTQEGSGDGPSSSVDWNRPEDVDPQGIYVISAPSIYAREVATPLFPPLHTGRAGQRQHLLFPYPSSILSVK

SEQ ID NO: 111 - protein, 626 aa, Artificial Sequence
  FLAG-tagged cyno DLL3 full length
MVSPRMSRLLSQTVILALIFIPQARPDYKDDDDKAGVFELQIHSFGPGPGPGAPRSPCSARGPCRLFFRVCLKPGLSEEAAESPCALGAALSARGPVYTEQPEAPAPDLPLPNGLLQVPFRDAWPGTFSLIIETWREELGDQIGGPAWSLLARVTRRRRLAAGGPWARDIQRAGAWELRFSYRARCELPAVGTACTRLCRPRSAPSRCGPGLRPCAPLEDECEAPPVCRAGCSLEHGFCEQPGECRCLEGWTGPLCMVPVSTSSCLGLRGPSSTTTGCLVPGPGPCDGNPCANGGSCSETPGSFECTCPRGFYGLRCEVSGVTCADGPCFNGGLCVGGADPDSAYICHCPPGFQGSNCEKRVDRCSLQPCRNGGLCLDLGHALRCRCRAGFAGPRCEHDLDDCAGRACANGGTCVEGGGAHRCSCALGFGGRNCRERADPCAARPCAHGGRCYAHFSGLVCACAPGYMGARCEFPVHPDGVSALPAAPPGLRPGDPQRYLLPPALGLLVAAGVAGAALLLVHVRRRGHAQDAGSRLLAGTPEPSVHALPDALNNLRTQEGPGDVPSSSVDWNRPEDVDSRGIYVISAPSIYAREVAMPLFPPLHTGRAGQRQNLLFPFPSSILSVK

SEQ ID NO: 112 - protein, 731 aa, Artificial Sequence
  FLAG-tagged human DLL1 full length
MGSRCALALAVLSALLCDYKDDDDKQVWSSGVFELKLQEFVNKKGLLGNRNCCRGGAGPPPCACRTFFRVCLKHYQASVSPEPPCTYGSAVTPVLGVDSFSLPDGGGADSAFSNPIRFPFGFTWPGTFSLIIEALHTDSPDDLATENPERLISRLATQRHLTVGEEWSQDLHSSGRTDLKYSYRFVCDEHYYGEGCSVFCRPRDDAFGHFTCGERGEKVCNPGWKGPYCTEPICLPGCDEQHGFCDKPGECKCRVGWQGRYCDECIRYPGCLHGTCQQPWQCNCQEGWGGLFCNQDLNYCTHHKPCKNGATCTNTGQGSYTCSCRPGYTGATCELGIDECDPSPCKNGGSCTDLENSYSCTCPPGFYGKICELSAMTCADGPCFNGGRCSDSPDGGYSCRCPVGYSGFNCEKKIDYCSSSPCSNGAKCVDLGDAYLCRCQAGFSGRHCDDNVDDCASSPCANGGTCRDGVNDFSCTCPPGYTGRNCSAPVSRCEHAPCHNGATCHERGHRYVCECARGYGGPNCQFLLPELPPGPAVVDLTEKLEGQGGPFPWVAVCAGVILVLMLLLGCAAVVVCVRLRLQKHRPPADPCRGETETMNNLANCQREKDISVSIIGATQIKNTNKKADFHGDHSADKNGFKARYPAVDYNLVQDLKGDDTAVRDAHSKRDTKCQPQGSSGEEKGTPTTLRGGEASERKRPDSGCSTSKDTKYQSVYVISEEKDECVIATEV

SEQ ID NO: 113 - protein, 693 aa, Artificial Sequence
  FLAG-tagged human DLL4 full length
MAAASRSASGWALLLLVALWQQRAAGDYKDDDDKSGVFQLQLQEFINERGVLASGRPCEPGCRTFFRVCLKHFQAVVSPGPCTFGTVSTPVLGTNSFAVRDDSSGGGRNPLQLPFNFTWPGTFSLIIEAWHAPGDDLRPEALPPDALISKIAIQGSLAVGQNWLLDEQTSTLTRLRYSYRVICSDNYYGDNCSRLCKKRNDHFGHYVCQPDGNLSCLPGWTGEYCQQPICLSGCHEQNGYCSKPAECLCRPGWQGRLCNECIPHNGCRHGTCSTPWQCTCDEGWGGLFCDQDLNYCTHHSPCKNGATCSNSGQRSYTCTCRPGYTGVDCELELSECDSNPCRNGGSCKDQEDGYHCLCPPGYYGLHCEHSTLSCADSPCFNGGSCRERNQGANYACECPPNFTGSNCEKKVDRCTSNPCANGGQCLNRGPSRMCRCRPGFTGTYCELHVSDCARNPCAHGGTCHDLENGLMCTCPAGFSGRRCEVRTSIDACASSPCFNRATCYTDLSTDTFVCNCPYGFVGSRCEFPVGLPPSFPWVAVSLGVGLAVLLVLLGMVAVAVRQLRLRRPDDGSREAMNNLSDFQKDNLIPAAQLKNTNQKKELEVDCGLDKSNCGKQQNHTLDYNLAPGPLGRGTMPGKFPHSDKSLGEKAPLRLHSEKPECRISAICSPRDSMYQSVCLISEERNECVIATEV

SEQ ID NO: 114 - protein, 8 aa, Artificial Sequence
  FLAG tag
DYKDDDDK

SEQ ID NO: 115 - protein, 21 aa, Artificial Sequence
  Vk leader
METDTLLLWVLLLWVPGSTGD

SEQ ID NO: 116 - protein, 16 aa, Artificial Sequence
  6His-myc tag
HHHHHHEQKLISEEDL

SEQ ID NO: 117 - protein, 6 aa, Artificial Sequence
  Ser/Gly linker
SGGGGS

SEQ ID NO: 118 - protein, 23 aa, Artificial Sequence
  EpCAM transmembrane domain
AGVIAVIVVVVIAVVAGIVVLVI

SEQ ID NO: 119 - protein, 26 aa, Artificial Sequence
  EpCAM intracellular domain
SRKKRMAKYEKAEIKEMGEMHRELNA

SEQ ID NO: 120 - protein, 34 aa, Artificial Sequence
  EGF1
APLVCRAGCSPEHGFCEQPGECRCLEGWTGPLCT

SEQ ID NO: 121 - protein, 95 aa, Artificial Sequence
  Hu DLL3 EGF 1+2
APLVCRAGCSPEHGFCEQPGECRCLEGWTGPLCTVPVSTSSCLSPRGPSSATTGCLVPGPGPCDGNPCANGGSCSETPRSFECTCPRGFYGLRCE

SEQ ID NO: 122 - protein, 37 aa, Artificial Sequence
  EGF2
GPGPCDGNPCANGGSCSETPRSFECTCPRGFYGLRCE

SEQ ID NO: 123 - protein, 78 aa, Artificial Sequence
  Hu DLL3 EGF 2+3
GPGPCDGNPCANGGSCSETPRSFECTCPRGFYGLRCEVSGVTCADGPCFNGGLCVGGADPDSAYICHCPPGFQGSNCE

SEQ ID NO: 124 - protein, 40 aa, Artificial Sequence
  EGF3
SGVTCADGPCFNGGLCVGGADPDSAYICHCPPGFQGSNCE

SEQ ID NO: 125 - protein, 78 aa, Artificial Sequence
  Hu DLL3 EGF 3+4
SGVTCADGPCFNGGLCVGGADPDSAYICHCPPGFQGSNCEKRVDRCSLQPCRNGGLCLDLGHALRCRCRAGFAGPRCE

SEQ ID NO: 126 - protein, 37 aa, Artificial Sequence
  EGF4
RVDRCSLQPCRNGGLCLDLGHALRCRCRAGFAGPRCE

SEQ ID NO: 127 - protein, 75 aa, Artificial Sequence
  Hu DLL3 EGF 4+5
RVDRCSLQPCRNGGLCLDLGHALRCRCRAGFAGPRCEHDLDDCAGRACANGGTCVEGGGAHRCSCALGFGGRDCR

SEQ ID NO: 128 - protein, 37 aa, Artificial Sequence
  EGF5
DLDDCAGRACANGGTCVEGGGAHRCSCALGFGGRDCR

SEQ ID NO: 129 - protein, 73 aa, Artificial Sequence
  Hu DLL3 EGF 5+6
DDCAGRACANGGTCVEGGGAHRCSCALGFGGRDCRERADPCAARPCAHGGRCYAHFSGLVCACAPGYMGARCE

SEQ ID NO: 130 - protein, 37 aa, Artificial Sequence
  EGF6
RADPCAARPCAHGGRCYAHFSGLVCACAPGYMGARCE

SEQ ID NO: 131 - protein, 64 aa, Artificial Sequence
  Hu DLL3 EGF6-membrane proximal peptide
RADPCAARPCAHGGRCYAHFSGLVCACAPGYMGARCEFPVHPDGASALPAAPPGLRPGDPQRYL

SEQ ID NO: 132 - protein, 27 aa, Artificial Sequence
  Membrane proximal peptide
FPVHPDGASALPAAPPGLRPGDPQRYL

SEQ ID NO: 133 - protein, 12 aa, Artificial Sequence
  DLL3#7 LCCDR1
RASQSVNSNFLA

SEQ ID NO: 134 - protein, 7 aa, Artificial Sequence
  DLL3#7 LCCDR2
GTSSRAT

SEQ ID NO: 135 - protein, 9 aa, Artificial Sequence
  DLL3#7 LCCDR3
QQYGSSPWT

SEQ ID NO: 136 - protein, 10 aa, Artificial Sequence
  DLL3#7 HCCDR1
GFTFSSYGMF

SEQ ID NO: 137 - protein, 17 aa, Artificial Sequence
  DLL3#7 HCCDR2
VIWLDGDDEDYVDSVKG

SEQ ID NO: 138 - protein, 4 aa, Artificial Sequence
  DLL3#7 HCCDR3
VLDY

SEQ ID NO: 139 - protein, 17 aa, Artificial Sequence
  DLL3#8 LCCDR1
KSSQSVLDTSNNKNYLV

SEQ ID NO: 140 - protein, 7 aa, Artificial Sequence
  DLL3#8 LCCDR2
WASTRES

SEQ ID NO: 141 - protein, 9 aa, Artificial Sequence
  DLL3#8 LCCDR3
QHYYNSPYT

SEQ ID NO: 142 - protein, 10 aa, Artificial Sequence
  DLL3#8 HCCDR1
GYTFTDYYMH

SEQ ID NO: 143 - protein, 17 aa, Artificial Sequence
  DLL3#8 HCCDR2
WINPNSGGTNYEQKFQG

SEQ ID NO: 144 - protein, 9 aa, Artificial Sequence
  DLL3#8 HCCDR3
DAVVIPMDY

SEQ ID NO: 145 - protein, 12 aa, Artificial Sequence
  DLL3#9 LCCDR1
RASQSISRSYLA

SEQ ID NO: 146 - protein, 7 aa, Artificial Sequence
  DLL3#9 LCCDR2
GASSRAT

SEQ ID NO: 147 - protein, 9 aa, Artificial Sequence
  DLL3#9 LCCDR3
QQYGTSPIT

SEQ ID NO: 148 - protein, 10 aa, Artificial Sequence
  DLL3#9 HCCDR1
GGSISSYYWS

SEQ ID NO: 149 - protein, 16 aa, Artificial Sequence
  DLL3#9 HCCDR2
YRYYSGNTNYNPSLKS

SEQ ID NO: 150 - protein, 10 aa, Artificial Sequence
  DLL3#9 HCCDR3
IGVAGFYFDY

SEQ ID NO: 151 - protein, 12 aa, Artificial Sequence
  DLL3#10 LCCDR1
RASQSLNSIFLA

SEQ ID NO: 152 - protein, 7 aa, Artificial Sequence
  DLL3#10 LCCDR2
GASSRAT

SEQ ID NO: 153 - protein, 9 aa, Artificial Sequence
  DLL3#10 LCCDR3
QQYGGSMNT

SEQ ID NO: 154 - protein, 10 aa, Artificial Sequence
  DLL3#10 HCCDR1
GYTFTGYYMH

SEQ ID NO: 155 - protein, 17 aa, Artificial Sequence
  DLL3#10 HCCDR2
WINPNSGGTIFAQRFQG

SEQ ID NO: 156 - protein, 12 aa, Artificial Sequence
  DLL3#10 HCCDR3
DFGDTVGNAFDI

SEQ ID NO: 157 - protein, 10 aa, Artificial Sequence
  DLL3#11 LCCDR1
SASSSVTYIH

SEQ ID NO: 158 - protein, 7 aa, Artificial Sequence
  DLL3#11 LCCDR2
RTSYLAS

SEQ ID NO: 159 - protein, 9 aa, Artificial Sequence
  DLL3#11 LCCDR3
QQRSSYPRT

SEQ ID NO: 160 - protein, 10 aa, Artificial Sequence
  DLL3#11 HCCDR1
GYAFSDYWIT

SEQ ID NO: 161 - protein, 17 aa, Artificial Sequence
  DLL3#11 HCCDR2
DIYPGSGSTKSSEKFKN

SEQ ID NO: 162 - protein, 11 aa, Artificial Sequence
  DLL3#11 HCCDR3
LYYYGSHYLDT

SEQ ID NO: 163 - protein, 10 aa, Artificial Sequence
  DLL3#12 LCCDR1
SASSSVTYIH

SEQ ID NO: 164 - protein, 7 aa, Artificial Sequence
  DLL3#12 LCCDR2
RTSYLAS

SEQ ID NO: 165 - protein, 9 aa, Artificial Sequence
  DLL3#12 LCCDR3
QQRSSYPRT

SEQ ID NO: 166 - protein, 10 aa, Artificial Sequence
  DLL3#12 HCCDR1
GYAFSDYWIT

SEQ ID NO: 167 - protein, 17 aa, Artificial Sequence
  DLL3#12 HCCDR2
DIYPGSGSTKSSEKFKN

SEQ ID NO: 168 - protein, 11 aa, Artificial Sequence
  DLL3#12 HCCDR3
LYYYGSYYLDT

SEQ ID NO: 169 - protein, 16 aa, Artificial Sequence
  DLL3#13 LCCDR1
RSSQSIVHSNGNTYLE

SEQ ID NO: 170 - protein, 7 aa, Artificial Sequence
  DLL3#13 LCCDR2
KVSNRFS

SEQ ID NO: 171 - protein, 9 aa, Artificial Sequence
  DLL3#13 LCCDR3
FQGSHVPYT

SEQ ID NO: 172 - protein, 10 aa, Artificial Sequence
  DLL3#13 HCCDR1
GYTFTNYGVT

SEQ ID NO: 173 - protein, 17 aa, Artificial Sequence
  DLL3#13 HCCDR2
WINTYSGAPTYADDFNG

SEQ ID NO: 174 - protein, 11 aa, Artificial Sequence
  DLL3#13 HCCDR3
LDDYDLYYFDY

SEQ ID NO: 175 - protein, 15 aa, Artificial Sequence
  DLL3#14 LCCDR1
KASQSVDYDGDSYMN

SEQ ID NO: 176 - protein, 7 aa, Artificial Sequence
  DLL3#14 LCCDR2
AASTLES

SEQ ID NO: 177 - protein, 9 aa, Artificial Sequence
  DLL3#14 LCCDR3
QQSDEDPWT

SEQ ID NO: 178 - protein, 10 aa, Artificial Sequence
  DLL3#14 HCCDR1
GYTFTDYYIH

SEQ ID NO: 179 - protein, 17 aa, Artificial Sequence
  DLL3#14 HCCDR2
YIYPGNSYTAYNQKFKD

SEQ ID NO: 180 - protein, 8 aa, Artificial Sequence
  DLL3#14 HCCDR3
SGGSAMDY

SEQ ID NO: 181 - protein, 15 aa, Artificial Sequence
  DLL3#15 LCCDR1
KASQSVDYDGDSYLN

SEQ ID NO: 182 - protein, 7 aa, Artificial Sequence
  DLL3#15 LCCDR2
AASNLES

SEQ ID NO: 183 - protein, 9 aa, Artificial Sequence
  DLL3#15 LCCDR3
QQSSEDPRT

SEQ ID NO: 184 - protein, 10 aa, Artificial Sequence
  DLL3#15 HCCDR1
GYTFTNYGMN

SEQ ID NO: 185 - protein, 17 aa, Artificial Sequence
  DLL3#15 HCCDR2
WINTYTGEPTYADDFKG

SEQ ID NO: 186 - protein, 12 aa, Artificial Sequence
  DLL3#15 HCCDR3
FHFSSNGDAMDN

SEQ ID NO: 187 - protein, 11 aa, Artificial Sequence
  DLL3#16 LCCDR1
RASQSVSDWLA

SEQ ID NO: 188 - protein, 7 aa, Artificial Sequence
  DLL3#16 LCCDR2
RASSLES

SEQ ID NO: 189 - protein, 9 aa, Artificial Sequence
  DLL3#16 LCCDR3
QLYNSYSPT

SEQ ID NO: 190 - protein, 10 aa, Artificial Sequence
  DLL3#16 HCCDR1
GFTFSSYWMT

SEQ ID NO: 191 - protein, 17 aa, Artificial Sequence
  DLL3#16 HCCDR2
NIKEDGSEKYYVDSVKG

SEQ ID NO: 192 - protein, 7 aa, Artificial Sequence
  DLL3#16 HCCDR3
DWGYFDY

SEQ ID NO: 193 - protein, 11 aa, Artificial Sequence
  DLL3#17 LCCDR1
RASENIYYSLA

SEQ ID NO: 194 - protein, 7 aa, Artificial Sequence
  DLL3#17 LCCDR2
NTNSLED

SEQ ID NO: 195 - protein, 9 aa, Artificial Sequence
  DLL3#17 LCCDR3
KQAYDFPLT

SEQ ID NO: 196 - protein, 10 aa, Artificial Sequence
  DLL3#17 HCCDR1
GYTFISYYIH

SEQ ID NO: 197 - protein, 17 aa, Artificial Sequence
  DLL3#17 HCCDR2
WIYPGDGSTNNNEKFKG

SEQ ID NO: 198 - protein, 8 aa, Artificial Sequence
  DLL3#17 HCCDR3
GEGNAMDD

SEQ ID NO: 199 - protein, 11 aa, Artificial Sequence
  DLL3#18 LCCDR1
RASENIYYSLA

SEQ ID NO: 200 - protein, 7 aa, Artificial Sequence
  DLL3#18 LCCDR2
NANSLED

SEQ ID NO: 201 - protein, 9 aa, Artificial Sequence
  DLL3#18 LCCDR3
KQAYDVPLT

SEQ ID NO: 202 - protein, 10 aa, Artificial Sequence
  DLL3#18 HCCDR1
GYTFTAYFIH

SEQ ID NO: 203 - protein, 17 aa, Artificial Sequence
  DLL3#18 HCCDR2
YIDPFNDDTNYNVKFKG

SEQ ID NO: 204 - protein, 8 aa, Artificial Sequence
  DLL3#18 HCCDR3
GTSATLDY

SEQ ID NO: 205 - protein, 108 aa, Artificial Sequence
  DLL3#7 VL
EIVLTQSPDTLSLSPGERATLSCRASQSVNSNFLAWYQQKPGQTPRLLIFGTSSRATGIPDRFSGSGSGTDFTLTISRLEPEDFAVYYCQQYGSSPWTFGQGTKVEIR

SEQ ID NO: 206 - protein, 113 aa, Artificial Sequence
  DLL3#7 VH
QVQLVESGGGVVQPGRSLRLSCAASGFTFSSYGMFWVRQAPGKGLEWVAVIWLDGDDEDYVDSVKGRFTISRDDSKNTLYLQMNSLRVDDTAIYYCARVLDYWGQGTLVTVSS

SEQ ID NO: 207 - protein, 113 aa, Artificial Sequence
  DLL3#8 VL
DIVMAQSPDSLAVSLGERATINCKSSQSVLDTSNNKNYLVWYQQKPGQPPKLLIYWASTRESGVPDRFSGSGSGTDFTLTISSLQAEDVAVYYCQHYYNSPYTFGQGTKLEIK

SEQ ID NO: 208 - protein, 118 aa, Artificial Sequence
  DLL3#8 VH
QVQLVQSGAEVKKPGASVKVSCKASGYTFTDYYMHWVRQAPGQGLEWMGWINPNSGGTNYEQKFQGRVTMTRDTSISTAYMELNRLRSDDTAVYYCTRDAVVIPMDYWGQGTLVTVSS

SEQ ID NO: 209 - protein, 108 aa, Artificial Sequence
  DLL3#9 VL
EIVLTQSPGTLSLSPGERATLSCRASQSISRSYLAWYQQKPGQAPRLLIYGASSRATGIPDRFSGSGSGTDFTLTISRLEPEDFAVYYCQQYGTSPITFGQGTRLEIK

SEQ ID NO: 210 - protein, 118 aa, Artificial Sequence
  DLL3#9 VH
QVHLQESGPGLVKPSETLSLTCTVSGGSISSYYWSWIRQTPGKGLDWIGYRYYSGNTNYNPSLKSRVTISLDMSNNQFSLKLSSVTAADTAIYYCASIGVAGFYFDYWGQGTLVTVSS

SEQ ID NO: 211 - protein, 108 aa, Artificial Sequence
  DLL3#10 VL
EIVLTQSPGTLSLSPGERATLSCRASQSLNSIFLAWYQQKPGQAPWLLIYGASSRATGIPDRFSGSGSGTDFTLTISRLEPEDFAVYFCQQYGGSMNTFGQGTKLEIK

SEQ ID NO: 212 - protein, 121 aa, Artificial Sequence
  DLL3#10 VH
QVQLVQSGAEVKKPGASVKVSCKASGYTFTGYYMHWVRLAPGQGLEWMGWINPNSGGTIFAQRFQGRVTMTRDTSISTVYMDLNRLRSDDTAVYYCARDFGDTVGNAFDIWGQGTMVTVSS

SEQ ID NO: 213 - protein, 106 aa, Artificial Sequence
  DLL3#11 VL
QIVLTQSPAIMSASPGEKVTITCSASSSVTYIHWFQQNPGTSPKLWIYRTSYLASGVPARFSGSGSGTSYSLTISRMEAEDAATYYCQQRSSYPRTFGGGTKLEIK

SEQ ID NO: 214 - protein, 120 aa, Artificial Sequence
  DLL3#11 VH
QVQLQQPGAELVQPGSSVKMSCKASGYAFSDYWITWVKQRPGQGLEWIGDIYPGSGSTKSSEKFKNKATLTADTSSSKAYIQFSSLTPEDSAVYYCVSLYYYGSHYLDTWGQGTTLTVSS

SEQ ID NO: 215 - protein, 106 aa, Artificial Sequence
  DLL3#12 VL
QVVLTQSPAIMSASPGEKVTITCSASSSVTYIHWFQQNPGTSPKLWIYRTSYLASGVPARFSGSGSGTSYSLTISRMEAEDAATYYCQQRSSYPRTFGGGTKLEIK

SEQ ID NO: 216 - protein, 120 aa, Artificial Sequence
  DLL3#12 VH
QVQLQQPGAEFVQPGSSVKMSCKASGYAFSDYWITWVKQRPGQGLEWIGDIYPGSGSTKSSEKFKNRATLTADTSSSTAYIQFSSLTPEDSAVYYCVSLYYYGSYYLDTWGQGTTLTVSS

SEQ ID NO: 217 - protein, 112 aa, Artificial Sequence
  DLL3#13 VL
DVLMTQTPLSLPVSLGDQAAISCRSSQSIVHSNGNTYLEWYLQKPGQSPKVLIYKVSNRFSGVPDRFSGSGSGTDFTLKISRVEAEDLGVYYCFQGSHVPYTFGGGTKLEIK

SEQ ID NO: 218 - protein, 120 aa, Artificial Sequence
  DLL3#13 VH
QIQLVQSGPELKKPGETVKISCKASGYTFTNYGVTWVKQAPGKGLKWMGWINTYSGAPTYADDFNGRFALSLETSASTAYLQINNLKNEDTATYFCARLDDYDLYYFDYWGQGTALTVSS

SEQ ID NO: 219 - protein, 111 aa, Artificial Sequence
  DLL3#14 VL
DIVLTQSPASLSVSLGQRATISCKASQSVDYDGDSYMNWYQQKPGQPPKLLIYAASTLESGIPARFSGSGSGTDFTLNIHPVEEEDAATYYCQQSDEDPWTFGGGTKLEIK

SEQ ID NO: 220 - protein, 115 aa, Artificial Sequence
  DLL3#14 VH
QIQLQQSGPELVKPGVKISCKASGYTFTDYYIHWMKQRPGQGLEWIGYIYPGNSYTAYNQKFKDKATLTADNPSSTAYMQLSSLTSEDSAVYFCARSGGSAMDYWGQGTSVTVSS

SEQ ID NO: 221 - protein, 111 aa, Artificial Sequence
  DLL3#15 VL
DIVLTQSPASLAVSLGQRATISCKASQSVDYDGDSYLNWYQQKPGQPPKLLIYAASNLESGIPARFSGSGSGTDFTLNIHPVEEEDAATYYCQQSSEDPRTFGGGTKLEIK

SEQ ID NO: 222 - protein, 121 aa, Artificial Sequence
  DLL3#15 VH
QIQLVQSGPELKKPGETVKISCKASGYTFTNYGMNWVKQAPGKGLKWMGWINTYTGEPTYADDFKGRFAFSLETSASTAYLQINNLKNEDMATYFCTKFHFSSNGDAMDNWGQGTSVTVSS

SEQ ID NO: 223 - protein, 107 aa, Artificial Sequence
  DLL3#16 VL
DIQMTQSPSTLSASVGDRVTITCRASQSVSDWLAWYQQKPGKAPKFLIYRASSLESGVPSRFSGSGSGTEFTLTISSLQPADFATYYCQLYNSYSPTFGQGTKVEIK

SEQ ID NO: 224 - protein, 116 aa, Artificial Sequence
  DLL3#16 VH
EVHLVESGGGLVQPGGSLRLSCAASGFTFSSYWMTWVRQAPGKGLEWVANIKEDGSEKYYVDSVKGRFTISRDNAKNSLYLQMNSLRAEDTALYYCARDWGYFDYWGQGTLVTVSS

SEQ ID NO: 225 - protein, 107 aa, Artificial Sequence
  DLL3#17 VL
DIQMTQSPASLAASVGETVTITCRASENIYYSLAWYQQKQGKSPQLLIYNTNSLEDGVPSRFSGSGSGTQYSMKINSMQPEDTATYFCKQAYDFPLTFGAGTKLELK

SEQ ID NO: 226 - protein, 117 aa, Artificial Sequence
  DLL3#17 VH
QIQLQQSGPEVVKPGASVKISCKASGYTFISYYIHWVKQRPGQGLEWIGWIYPGDGSTNNNEKFKGKTTLTADKSSSTAYMLLSSLTSEDSAVYFCARGEGNAMDDWGQGTSVTVSS

SEQ ID NO: 227 - protein, 107 aa, Artificial Sequence
  DLL3#18 VL
DIQMTQSPASLAASVGETVTITCRASENIYYSLAWYQQKQGKSPQLLIYNANSLEDGVPSRFSGSGSGTQYSMKINNMQPEDTATYFCKQAYDVPLTFGAGTKLELK

SEQ ID NO: 228 - protein, 117 aa, Artificial Sequence
  DLL3#18 VH
QVQLQQSGPDLVKPGASVKMSCEASGYTFTAYFIHWVKQKPGQGLEWIGYIDPFNDDTNYNVKFKGKATLTSDTSSSIAYMELSSLTSEDSSFYYCARGTSATLDYWGHGTTLTVSS

SEQ ID NO: 229 - protein, 469 aa, Artificial Sequence
  DLL3#7 scFab
EIVLTQSPDTLSLSPGERATLSCRASQSVNSNFLAWYQQKPGQTPRLLIFGTSSRATGIPDRFSGSGSGTDFTLTISRLEPEDFAVYYCQQYGSSPWTFGQGTKVEIRRTVAAPSVFIFPPSDEQLKSGTASVVCLLNNFYPREAKVQWKVDNALQSGNSQESVTEQDSKDSTYSLSSTLTLSKADYEKHKVYACEVTHQGLSSPVTKSFNRGECGGGGSEGKSSGSGSESKSTEGKSSGSGSESKSTGGGGSQVQLVESGGGVVQPGRSLRLSCAASGFTFSSYGMFWVRQAPGKGLEWVAVIWLDGDDEDYVDSVKGRFTISRDDSKNTLYLQMNSLRVDDTAIYYCARVLDYWGQGTLVTVSSASTKGPSVFPLAPSSKSTSGGTAALGCLVKDYFPEPVTVSWNSGALTSGVHTFPAVLQSSGLYSLSSVVTVPSSSLGTQTYICNVNHKPSNTKVDKRVEPKSC

SEQ ID NO: 230 - protein, 479 aa, Artificial Sequence
  DLL3#8 scFab
DIVMAQSPDSLAVSLGERATINCKSSQSVLDTSNNKNYLVWYQQKPGQPPKLLIYWASTRESGVPDRFSGSGSGTDFTLTISSLQAEDVAVYYCQHYYNSPYTFGQGTKLEIKRTVAAPSVFIFPPSDEQLKSGTASVVCLLNNFYPREAKVQWKVDNALQSGNSQESVTEQDSKDSTYSLSSTLTLSKADYEKHKVYACEVTHQGLSSPVTKSFNRGECGGGGSEGKSSGSGSESKSTEGKSSGSGSESKSTGGGGSQVQLVQSGAEVKKPGASVKVSCKASGYTFTDYYMHWVRQAPGQGLEWMGWINPNSGGTNYEQKFQGRVTMTRDTSISTAYMELNRLRSDDTAVYYCTRDAVVIPMDYWGQGTLVTVSSASTKGPSVFPLAPSSKSTSGGTAALGCLVKDYFPEPVTVSWNSGALTSGVHTFPAVLQSSGLYSLSSVVTVPSSSLGTQTYICNVNHKPSNTKVDKRVEPKSC

SEQ ID NO: 231 - protein, 474 aa, Artificial Sequence
  DLL3#9 scFab
EIVLTQSPGTLSLSPGERATLSCRASQSISRSYLAWYQQKPGQAPRLLIYGASSRATGIPDRFSGSGSGTDFTLTISRLEPEDFAVYYCQQYGTSPITFGQGTRLEIKRTVAAPSVFIFPPSDEQLKSGTASVVCLLNNFYPREAKVQWKVDNALQSGNSQESVTEQDSKDSTYSLSSTLTLSKADYEKHKVYACEVTHQGLSSPVTKSFNRGECGGGGSEGKSSGSGSESKSTEGKSSGSGSESKSTGGGGSQVHLQESGPGLVKPSETLSLTCTVSGGSISSYYWSWIRQTPGKGLDWIGYRYYSGNTNYNPSLKSRVTISLDMSNNQFSLKLSSVTAADTAIYYCASIGVAGFYFDYWGQGTLVTVSSASTKGPSVFPLAPSSKSTSGGTAALGCLVKDYFPEPVTVSWNSGALTSGVHTFPAVLQSSGLYSLSSVVTVPSSSLGTQTYICNVNHKPSNTKVDKRVEPKSC

SEQ ID NO: 232 - protein, 477 aa, Artificial Sequence
  DLL3#10 scFab
EIVLTQSPGTLSLSPGERATLSCRASQSLNSIFLAWYQQKPGQAPWLLIYGASSRATGIPDRFSGSGSGTDFTLTISRLEPEDFAVYFCQQYGGSMNTFGQGTKLEIKRTVAAPSVFIFPPSDEQLKSGTASVVCLLNNFYPREAKVQWKVDNALQSGNSQESVTEQDSKDSTYSLSSTLTLSKADYEKHKVYACEVTHQGLSSPVTKSFNRGECGGGGSEGKSSGSGSESKSTEGKSSGSGSESKSTGGGGSQVQLVQSGAEVKKPGASVKVSCKASGYTFTGYYMHWVRLAPGQGLEWMGWINPNSGGTIFAQRFQGRVTMTRDTSISTVYMDLNRLRSDDTAVYYCARDFGDTVGNAFDIWGQGTMVTVSSASTKGPSVFPLAPSSKSTSGGTAALGCLVKDYFPEPVTVSWNSGALTSGVHTFPAVLQSSGLYSLSSVVTVPSSSLGTQTYICNVNHKPSNTKVDKRVEPKSC

SEQ ID NO: 233 - protein, 474 aa, Artificial Sequence
  DLL3#11 scFab
QIVLTQSPAIMSASPGEKVTITCSASSSVTYIHWFQQNPGTSPKLWIYRTSYLASGVPARFSGSGSGTSYSLTISRMEAEDAATYYCQQRSSYPRTFGGGTKLEIKRTVAAPSVFIFPPSDEQLKSGTASVVCLLNNFYPREAKVQWKVDNALQSGNSQESVTEQDSKDSTYSLSSTLTLSKADYEKHKVYACEVTHQGLSSPVTKSFNRGECGGGGSEGKSSGSGSESKSTEGKSSGSGSESKSTGGGGSQVQLQQPGAELVQPGSSVKMSCKASGYAFSDYWITWVKQRPGQGLEWIGDIYPGSGSTKSSEKFKNKATLTADTSSSKAYIQFSSLTPEDSAVYYCVSLYYYGSHYLDTWGQGTTLTVSSASTKGPSVFPLAPSSKSTSGGTAALGCLVKDYFPEPVTVSWNSGALTSGVHTFPAVLQSSGLYSLSSVVTVPSSSLGTQTYICNVNHKPSNTKVDKRVEPKSC

SEQ ID NO: 234 - protein, 474 aa, Artificial Sequence
  DLL3#12 scFab
QVVLTQSPAIMSASPGEKVTITCSASSSVTYIHWFQQNPGTSPKLWIYRTSYLASGVPARFSGSGSGTSYSLTISRMEAEDAATYYCQQRSSYPRTFGGGTKLEIKRTVAAPSVFIFPPSDEQLKSGTASVVCLLNNFYPREAKVQWKVDNALQSGNSQESVTEQDSKDSTYSLSSTLTLSKADYEKHKVYACEVTHQGLSSPVTKSFNRGECGGGGSEGKSSGSGSESKSTEGKSSGSGSESKSTGGGGSQVQLQQPGAEFVQPGSSVKMSCKASGYAFSDYWITWVKQRPGQGLEWIGDIYPGSGSTKSSEKFKNRATLTADTSSSTAYIQFSSLTPEDSAVYYCVSLYYYGSYYLDTWGQGTTLTVSSASTKGPSVFPLAPSSKSTSGGTAALGCLVKDYFPEPVTVSWNSGALTSGVHTFPAVLQSSGLYSLSSVVTVPSSSLGTQTYICNVNHKPSNTKVDKRVEPKSC

SEQ ID NO: 235 - protein, 480 aa, Artificial Sequence
  DLL3#13 scFab
DVLMTQTPLSLPVSLGDQAAISCRSSQSIVHSNGNTYLEWYLQKPGQSPKVLIYKVSNRFSGVPDRFSGSGSGTDFTLKISRVEAEDLGVYYCFQGSHVPYTFGGGTKLEIKRTVAAPSVFIFPPSDEQLKSGTASVVCLLNNFYPREAKVQWKVDNALQSGNSQESVTEQDSKDSTYSLSSTLTLSKADYEKHKVYACEVTHQGLSSPVTKSFNRGECGGGGSEGKSSGSGSESKSTEGKSSGSGSESKSTGGGGSQIQLVQSGPELKKPGETVKISCKASGYTFTNYGVTWVKQAPGKGLKWMGWINTYSGAPTYADDFNGRFALSLETSASTAYLQINNLKNEDTATYFCARLDDYDLYYFDYWGQGTALTVSSASTKGPSVFPLAPSSKSTSGGTAALGCLVKDYFPEPVTVSWNSGALTSGVHTFPAVLQSSGLYSLSSVVTVPSSSLGTQTYICNVNHKPSNTKVDKRVEPKSC

SEQ ID NO: 236 - protein, 474 aa, Artificial Sequence
  DLL3#14 scFab
DIVLTQSPASLSVSLGQRATISCKASQSVDYDGDSYMNWYQQKPGQPPKLLIYAASTLESGIPARFSGSGSGTDFTLNIHPVEEEDAATYYCQQSDEDPWTFGGGTKLEIKRTVAAPSVFIFPPSDEQLKSGTASVVCLLNNFYPREAKVQWKVDNALQSGNSQESVTEQDSKDSTYSLSSTLTLSKADYEKHKVYACEVTHQGLSSPVTKSFNRGECGGGGSEGKSSGSGSESKSTEGKSSGSGSESKSTGGGGSQIQLQQSGPELVKPGVKISCKASGYTFTDYYIHWMKQRPGQGLEWIGYIYPGNSYTAYNQKFKDKATLTADNPSSTAYMQLSSLTSEDSAVYFCARSGGSAMDYWGQGTSVTVSSASTKGPSVFPLAPSSKSTSGGTAALGCLVKDYFPEPVTVSWNSGALTSGVHTFPAVLQSSGLYSLSSVVTVPSSSLGTQTYICNVNHKPSNTKVDKRVEPKSC

SEQ ID NO: 237 - protein, 480 aa, Artificial Sequence
  DLL3#15 scFab
DIVLTQSPASLAVSLGQRATISCKASQSVDYDGDSYLNWYQQKPGQPPKLLIYAASNLESGIPARFSGSGSGTDFTLNIHPVEEEDAATYYCQQSSEDPRTFGGGTKLEIKRTVAAPSVFIFPPSDEQLKSGTASVVCLLNNFYPREAKVQWKVDNALQSGNSQESVTEQDSKDSTYSLSSTLTLSKADYEKHKVYACEVTHQGLSSPVTKSFNRGECGGGGSEGKSSGSGSESKSTEGKSSGSGSESKSTGGGGSQIQLVQSGPELKKPGETVKISCKASGYTFTNYGMNWVKQAPGKGLKWMGWINTYTGEPTYADDFKGRFAFSLETSASTAYLQINNLKNEDMATYFCTKFHFSSNGDAMDNWGQGTSVTVSSASTKGPSVFPLAPSSKSTSGGTAALGCLVKDYFPEPVTVSWNSGALTSGVHTFPAVLQSSGLYSLSSVVTVPSSSLGTQTYICNVNHKPSNTKVDKRVEPKSC

SEQ ID NO: 238 - protein, 471 aa, Artificial Sequence
  DLL3#16 scFab
DIQMTQSPSTLSASVGDRVTITCRASQSVSDWLAWYQQKPGKAPKFLIYRASSLESGVPSRFSGSGSGTEFTLTISSLQPADFATYYCQLYNSYSPTFGQGTKVEIKRTVAAPSVFIFPPSDEQLKSGTASVVCLLNNFYPREAKVQWKVDNALQSGNSQESVTEQDSKDSTYSLSSTLTLSKADYEKHKVYACEVTHQGLSSPVTKSFNRGECGGGGSEGKSSGSGSESKSTEGKSSGSGSESKSTGGGGSEVHLVESGGGLVQPGGSLRLSCAASGFTFSSYWMTWVRQAPGKGLEWVANIKEDGSEKYYVDSVKGRFTISRDNAKNSLYLQMNSLRAEDTALYYCARDWGYFDYWGQGTLVTVSSASTKGPSVFPLAPSSKSTSGGTAALGCLVKDYFPEPVTVSWNSGALTSGVHTFPAVLQSSGLYSLSSVVTVPSSSLGTQTYICNVNHKPSNTKVDKRVEPKSC

SEQ ID NO: 239 - protein, 472 aa, Artificial Sequence
  DLL3#17 scFab
DIQMTQSPASLAASVGETVTITCRASENIYYSLAWYQQKQGKSPQLLIYNTNSLEDGVPSRFSGSGSGTQYSMKINSMQPEDTATYFCKQAYDFPLTFGAGTKLELKRTVAAPSVFIFPPSDEQLKSGTASVVCLLNNFYPREAKVQWKVDNALQSGNSQESVTEQDSKDSTYSLSSTLTLSKADYEKHKVYACEVTHQGLSSPVTKSFNRGECGGGGSEGKSSGSGSESKSTEGKSSGSGSESKSTGGGGSQIQLQQSGPEVVKPGASVKISCKASGYTFISYYIHWVKQRPGQGLEWIGWIYPGDGSTNNNEKFKGKTTLTADKSSSTAYMLLSSLTSEDSAVYFCARGEGNAMDDWGQGTSVTVSSASTKGPSVFPLAPSSKSTSGGTAALGCLVKDYFPEPVTVSWNSGALTSGVHTFPAVLQSSGLYSLSSVVTVPSSSLGTQTYICNVNHKPSNTKVDKRVEPKSC

SEQ ID NO: 240 - protein, 472 aa, Artificial Sequence
  DLL3#18 scFab
DIQMTQSPASLAASVGETVTITCRASENIYYSLAWYQQKQGKSPQLLIYNANSLEDGVPSRFSGSGSGTQYSMKINNMQPEDTATYFCKQAYDVPLTFGAGTKLELKRTVAAPSVFIFPPSDEQLKSGTASVVCLLNNFYPREAKVQWKVDNALQSGNSQESVTEQDSKDSTYSLSSTLTLSKADYEKHKVYACEVTHQGLSSPVTKSFNRGECGGGGSEGKSSGSGSESKSTEGKSSGSGSESKSTGGGGSQVQLQQSGPDLVKPGASVKMSCEASGYTFTAYFIHWVKQKPGQGLEWIGYIDPFNDDTNYNVKFKGKATLTSDTSSSIAYMELSSLTSEDSSFYYCARGTSATLDYWGHGTTLTVSSASTKGPSVFPLAPSSKSTSGGTAALGCLVKDYFPEPVTVSWNSGALTSGVHTFPAVLQSSGLYSLSSVVTVPSSSLGTQTYICNVNHKPSNTKVDKRVEPKSC

SEQ ID NO: 241 - protein, 695 aa, Artificial Sequence
  DLL3#7 chain
EIVLTQSPDTLSLSPGERATLSCRASQSVNSNFLAWYQQKPGQTPRLLIFGTSSRATGIPDRFSGSGSGTDFTLTISRLEPEDFAVYYCQQYGSSPWTFGQGTKVEIRRTVAAPSVFIFPPSDEQLKSGTASVVCLLNNFYPREAKVQWKVDNALQSGNSQESVTEQDSKDSTYSLSSTLTLSKADYEKHKVYACEVTHQGLSSPVTKSFNRGECGGGGSEGKSSGSGSESKSTEGKSSGSGSESKSTGGGGSQVQLVESGGGVVQPGRSLRLSCAASGFTFSSYGMFWVRQAPGKGLEWVAVIWLDGDDEDYVDSVKGRFTISRDDSKNTLYLQMNSLRVDDTAIYYCARVLDYWGQGTLVTVSSASTKGPSVFPLAPSSKSTSGGTAALGCLVKDYFPEPVTVSWNSGALTSGVHTFPAVLQSSGLYSLSSVVTVPSSSLGTQTYICNVNHKPSNTKVDKRVEPKSCDKTHTCPPCPAPEAAGGPSVFLFPPKPKDTLMISRTPEVTCVVVDVSHEDPEVKFNWYVDGVEVHNAKTKPREEQYNSTYRVVSVLTVLHQDWLNGKEYKCKVSNKALPAPIEKTISKAKGQPREPQVYTLPPSREEMTKNQVSLWCLVKGFYPSDIAVEWESNGQPENNYKTTPPVLDSDGSFFLYSKLTVDKSRWQQGNVFSCSVMHEALHNHYTQKSLSLSPG

SEQ ID NO: 242 - protein, 705 aa, Artificial Sequence
  DLL3#8 chain
DIVMAQSPDSLAVSLGERATINCKSSQSVLDTSNNKNYLVWYQQKPGQPPKLLIYWASTRESGVPDRFSGSGSGTDFTLTISSLQAEDVAVYYCQHYYNSPYTFGQGTKLEIKRTVAAPSVFIFPPSDEQLKSGTASVVCLLNNFYPREAKVQWKVDNALQSGNSQESVTEQDSKDSTYSLSSTLTLSKADYEKHKVYACEVTHQGLSSPVTKSFNRGECGGGGSEGKSSGSGSESKSTEGKSSGSGSESKSTGGGGSQVQLVQSGAEVKKPGASVKVSCKASGYTFTDYYMHWVRQAPGQGLEWMGWINPNSGGTNYEQKFQGRVTMTRDTSISTAYMELNRLRSDDTAVYYCTRDAVVIPMDYWGQGTLVTVSSASTKGPSVFPLAPSSKSTSGGTAALGCLVKDYFPEPVTVSWNSGALTSGVHTFPAVLQSSGLYSLSSVVTVPSSSLGTQTYICNVNHKPSNTKVDKRVEPKSCDKTHTCPPCPAPEAAGGPSVFLFPPKPKDTLMISRTPEVTCVVVDVSHEDPEVKFNWYVDGVEVHNAKTKPREEQYNSTYRVVSVLTVLHQDWLNGKEYKCKVSNKALPAPIEKTISKAKGQPREPQVYTLPPSREEMTKNQVSLWCLVKGFYPSDIAVEWESNGQPENNYKTTPPVLDSDGSFFLYSKLTVDKSRWQQGNVFSCSVMHEALHNHYTQKSLSLSPG

SEQ ID NO: 243 - protein, 700 aa, Artificial Sequence
  DLL3#9 chain
EIVLTQSPGTLSLSPGERATLSCRASQSISRSYLAWYQQKPGQAPRLLIYGASSRATGIPDRFSGSGSGTDFTLTISRLEPEDFAVYYCQQYGTSPITFGQGTRLEIKRTVAAPSVFIFPPSDEQLKSGTASVVCLLNNFYPREAKVQWKVDNALQSGNSQESVTEQDSKDSTYSLSSTLTLSKADYEKHKVYACEVTHQGLSSPVTKSFNRGECGGGGSEGKSSGSGSESKSTEGKSSGSGSESKSTGGGGSQVHLQESGPGLVKPSETLSLTCTVSGGSISSYYWSWIRQTPGKGLDWIGYRYYSGNTNYNPSLKSRVTISLDMSNNQFSLKLSSVTAADTAIYYCASIGVAGFYFDYWGQGTLVTVSSASTKGPSVFPLAPSSKSTSGGTAALGCLVKDYFPEPVTVSWNSGALTSGVHTFPAVLQSSGLYSLSSVVTVPSSSLGTQTYICNVNHKPSNTKVDKRVEPKSCDKTHTCPPCPAPEAAGGPSVFLFPPKPKDTLMISRTPEVTCVVVDVSHEDPEVKFNWYVDGVEVHNAKTKPREEQYNSTYRVVSVLTVLHQDWLNGKEYKCKVSNKALPAPIEKTISKAKGQPREPQVYTLPPSREEMTKNQVSLWCLVKGFYPSDIAVEWESNGQPENNYKTTPPVLDSDGSFFLYSKLTVDKSRWQQGNVFSCSVMHEALHNHYTQKSLSLSPG

SEQ ID NO: 244 - protein, 703 aa, Artificial Sequence
  DLL3#10 chain
EIVLTQSPGTLSLSPGERATLSCRASQSLNSIFLAWYQQKPGQAPWLLIYGASSRATGIPDRFSGSGSGTDFTLTISRLEPEDFAVYFCQQYGGSMNTFGQGTKLEIKRTVAAPSVFIFPPSDEQLKSGTASVVCLLNNFYPREAKVQWKVDNALQSGNSQESVTEQDSKDSTYSLSSTLTLSKADYEKHKVYACEVTHQGLSSPVTKSFNRGECGGGGSEGKSSGSGSESKSTEGKSSGSGSESKSTGGGGSQVQLVQSGAEVKKPGASVKVSCKASGYTFTGYYMHWVRLAPGQGLEWMGWINPNSGGTIFAQRFQGRVTMTRDTSISTVYMDLNRLRSDDTAVYYCARDFGDTVGNAFDIWGQGTMVTVSSASTKGPSVFPLAPSSKSTSGGTAALGCLVKDYFPEPVTVSWNSGALTSGVHTFPAVLQSSGLYSLSSVVTVPSSSLGTQTYICNVNHKPSNTKVDKRVEPKSCDKTHTCPPCPAPEAAGGPSVFLFPPKPKDTLMISRTPEVTCVVVDVSHEDPEVKFNWYVDGVEVHNAKTKPREEQYNSTYRVVSVLTVLHQDWLNGKEYKCKVSNKALPAPIEKTISKAKGQPREPQVYTLPPSREEMTKNQVSLWCLVKGFYPSDIAVEWESNGQPENNYKTTPPVLDSDGSFFLYSKLTVDKSRWQQGNVFSCSVMHEALHNHYTQKSLSLSPG

SEQ ID NO: 245 - protein, 700 aa, Artificial Sequence
  DLL3#11 chain
QIVLTQSPAIMSASPGEKVTITCSASSSVTYIHWFQQNPGTSPKLWIYRTSYLASGVPARFSGSGSGTSYSLTISRMEAEDAATYYCQQRSSYPRTFGGGTKLEIKRTVAAPSVFIFPPSDEQLKSGTASVVCLLNNFYPREAKVQWKVDNALQSGNSQESVTEQDSKDSTYSLSSTLTLSKADYEKHKVYACEVTHQGLSSPVTKSFNRGECGGGGSEGKSSGSGSESKSTEGKSSGSGSESKSTGGGGSQVQLQQPGAELVQPGSSVKMSCKASGYAFSDYWITWVKQRPGQGLEWIGDIYPGSGSTKSSEKFKNKATLTADTSSSKAYIQFSSLTPEDSAVYYCVSLYYYGSHYLDTWGQGTTLTVSSASTKGPSVFPLAPSSKSTSGGTAALGCLVKDYFPEPVTVSWNSGALTSGVHTFPAVLQSSGLYSLSSVVTVPSSSLGTQTYICNVNHKPSNTKVDKRVEPKSCDKTHTCPPCPAPEAAGGPSVFLFPPKPKDTLMISRTPEVTCVVVDVSHEDPEVKFNWYVDGVEVHNAKTKPREEQYNSTYRVVSVLTVLHQDWLNGKEYKCKVSNKALPAPIEKTISKAKGQPREPQVYTLPPSREEMTKNQVSLWCLVKGFYPSDIAVEWESNGQPENNYKTTPPVLDSDGSFFLYSKLTVDKSRWQQGNVFSCSVMHEALHNHYTQKSLSLSPG

SEQ ID NO: 246 - protein, 700 aa, Artificial Sequence
  DLL3#12 chain
QVVLTQSPAIMSASPGEKVTITCSASSSVTYIHWFQQNPGTSPKLWIYRTSYLASGVPARFSGSGSGTSYSLTISRMEAEDAATYYCQQRSSYPRTFGGGTKLEIKRTVAAPSVFIFPPSDEQLKSGTASVVCLLNNFYPREAKVQWKVDNALQSGNSQESVTEQDSKDSTYSLSSTLTLSKADYEKHKVYACEVTHQGLSSPVTKSFNRGECGGGGSEGKSSGSGSESKSTEGKSSGSGSESKSTGGGGSQVQLQQPGAEFVQPGSSVKMSCKASGYAFSDYWITWVKQRPGQGLEWIGDIYPGSGSTKSSEKFKNRATLTADTSSSTAYIQFSSLTPEDSAVYYCVSLYYYGSYYLDTWGQGTTLTVSSASTKGPSVFPLAPSSKSTSGGTAALGCLVKDYFPEPVTVSWNSGALTSGVHTFPAVLQSSGLYSLSSVVTVPSSSLGTQTYICNVNHKPSNTKVDKRVEPKSCDKTHTCPPCPAPEAAGGPSVFLFPPKPKDTLMISRTPEVTCVVVDVSHEDPEVKFNWYVDGVEVHNAKTKPREEQYNSTYRVVSVLTVLHQDWLNGKEYKCKVSNKALPAPIEKTISKAKGQPREPQVYTLPPSREEMTKNQVSLWCLVKGFYPSDIAVEWESNGQPENNYKTTPPVLDSDGSFFLYSKLTVDKSRWQQGNVFSCSVMHEALHNHYTQKSLSLSPG

SEQ ID NO: 247 - protein, 706 aa, Artificial Sequence
  DLL3#13 chain
DVLMTQTPLSLPVSLGDQAAISCRSSQSIVHSNGNTYLEWYLQKPGQSPKVLIYKVSNRFSGVPDRFSGSGSGTDFTLKISRVEAEDLGVYYCFQGSHVPYTFGGGTKLEIKRTVAAPSVFIFPPSDEQLKSGTASVVCLLNNFYPREAKVQWKVDNALQSGNSQESVTEQDSKDSTYSLSSTLTLSKADYEKHKVYACEVTHQGLSSPVTKSFNRGECGGGGSEGKSSGSGSESKSTEGKSSGSGSESKSTGGGGSQIQLVQSGPELKKPGETVKISCKASGYTFTNYGVTWVKQAPGKGLKWMGWINTYSGAPTYADDFNGRFALSLETSASTAYLQINNLKNEDTATYFCARLDDYDLYYFDYWGQGTALTVSSASTKGPSVFPLAPSSKSTSGGTAALGCLVKDYFPEPVTVSWNSGALTSGVHTFPAVLQSSGLYSLSSVVTVPSSSLGTQTYICNVNHKPSNTKVDKRVEPKSCDKTHTCPPCPAPEAAGGPSVFLFPPKPKDTLMISRTPEVTCVVVDVSHEDPEVKFNWYVDGVEVHNAKTKPREEQYNSTYRVVSVLTVLHQDWLNGKEYKCKVSNKALPAPIEKTISKAKGQPREPQVYTLPPSREEMTKNQVSLWCLVKGFYPSDIAVEWESNGQPENNYKTTPPVLDSDGSFFLYSKLTVDKSRWQQGNVFSCSVMHEALHNHYTQKSLSLSPG

SEQ ID NO: 248 - protein, 700 aa, Artificial Sequence
  DLL3#14 chain
DIVLTQSPASLSVSLGQRATISCKASQSVDYDGDSYMNWYQQKPGQPPKLLIYAASTLESGIPARFSGSGSGTDFTLNIHPVEEEDAATYYCQQSDEDPWTFGGGTKLEIKRTVAAPSVFIFPPSDEQLKSGTASVVCLLNNFYPREAKVQWKVDNALQSGNSQESVTEQDSKDSTYSLSSTLTLSKADYEKHKVYACEVTHQGLSSPVTKSFNRGECGGGGSEGKSSGSGSESKSTEGKSSGSGSESKSTGGGGSQIQLQQSGPELVKPGVKISCKASGYTFTDYYIHWMKQRPGQGLEWIGYIYPGNSYTAYNQKFKDKATLTADNPSSTAYMQLSSLTSEDSAVYFCARSGGSAMDYWGQGTSVTVSSASTKGPSVFPLAPSSKSTSGGTAALGCLVKDYFPEPVTVSWNSGALTSGVHTFPAVLQSSGLYSLSSVVTVPSSSLGTQTYICNVNHKPSNTKVDKRVEPKSCDKTHTCPPCPAPEAAGGPSVFLFPPKPKDTLMISRTPEVTCVVVDVSHEDPEVKFNWYVDGVEVHNAKTKPREEQYNSTYRVVSVLTVLHQDWLNGKEYKCKVSNKALPAPIEKTISKAKGQPREPQVYTLPPSREEMTKNQVSLWCLVKGFYPSDIAVEWESNGQPENNYKTTPPVLDSDGSFFLYSKLTVDKSRWQQGNVFSCSVMHEALHNHYTQKSLSLSPG

SEQ ID NO: 249 - protein, 706 aa, Artificial Sequence
  DLL3#15 chain
DIVLTQSPASLAVSLGQRATISCKASQSVDYDGDSYLNWYQQKPGQPPKLLIYAASNLESGIPARFSGSGSGTDFTLNIHPVEEEDAATYYCQQSSEDPRTFGGGTKLEIKRTVAAPSVFIFPPSDEQLKSGTASVVCLLNNFYPREAKVQWKVDNALQSGNSQESVTEQDSKDSTYSLSSTLTLSKADYEKHKVYACEVTHQGLSSPVTKSFNRGECGGGGSEGKSSGSGSESKSTEGKSSGSGSESKSTGGGGSQIQLVQSGPELKKPGETVKISCKASGYTFTNYGMNWVKQAPGKGLKWMGWINTYTGEPTYADDFKGRFAFSLETSASTAYLQINNLKNEDMATYFCTKFHFSSNGDAMDNWGQGTSVTVSSASTKGPSVFPLAPSSKSTSGGTAALGCLVKDYFPEPVTVSWNSGALTSGVHTFPAVLQSSGLYSLSSVVTVPSSSLGTQTYICNVNHKPSNTKVDKRVEPKSCDKTHTCPPCPAPEAAGGPSVFLFPPKPKDTLMISRTPEVTCVVVDVSHEDPEVKFNWYVDGVEVHNAKTKPREEQYNSTYRVVSVLTVLHQDWLNGKEYKCKVSNKALPAPIEKTISKAKGQPREPQVYTLPPSREEMTKNQVSLWCLVKGFYPSDIAVEWESNGQPENNYKTTPPVLDSDGSFFLYSKLTVDKSRWQQGNVFSCSVMHEALHNHYTQKSLSLSPG

SEQ ID NO: 250 - protein, 697 aa, Artificial Sequence
  DLL3#16 chain
DIQMTQSPSTLSASVGDRVTITCRASQSVSDWLAWYQQKPGKAPKFLIYRASSLESGVPSRFSGSGSGTEFTLTISSLQPADFATYYCQLYNSYSPTFGQGTKVEIKRTVAAPSVFIFPPSDEQLKSGTASVVCLLNNFYPREAKVQWKVDNALQSGNSQESVTEQDSKDSTYSLSSTLTLSKADYEKHKVYACEVTHQGLSSPVTKSFNRGECGGGGSEGKSSGSGSESKSTEGKSSGSGSESKSTGGGGSEVHLVESGGGLVQPGGSLRLSCAASGFTFSSYWMTWVRQAPGKGLEWVANIKEDGSEKYYVDSVKGRFTISRDNAKNSLYLQMNSLRAEDTALYYCARDWGYFDYWGQGTLVTVSSASTKGPSVFPLAPSSKSTSGGTAALGCLVKDYFPEPVTVSWNSGALTSGVHTFPAVLQSSGLYSLSSVVTVPSSSLGTQTYICNVNHKPSNTKVDKRVEPKSCDKTHTCPPCPAPEAAGGPSVFLFPPKPKDTLMISRTPEVTCVVVDVSHEDPEVKFNWYVDGVEVHNAKTKPREEQYNSTYRVVSVLTVLHQDWLNGKEYKCKVSNKALPAPIEKTISKAKGQPREPQVYTLPPSREEMTKNQVSLWCLVKGFYPSDIAVEWESNGQPENNYKTTPPVLDSDGSFFLYSKLTVDKSRWQQGNVFSCSVMHEALHNHYTQKSLSLSPG

SEQ ID NO: 251 - protein, 698 aa, Artificial Sequence
  DLL3#17 chain
DIQMTQSPASLAASVGETVTITCRASENIYYSLAWYQQKQGKSPQLLIYNTNSLEDGVPSRFSGSGSGTQYSMKINSMQPEDTATYFCKQAYDFPLTFGAGTKLELKRTVAAPSVFIFPPSDEQLKSGTASVVCLLNNFYPREAKVQWKVDNALQSGNSQESVTEQDSKDSTYSLSSTLTLSKADYEKHKVYACEVTHQGLSSPVTKSFNRGECGGGGSEGKSSGSGSESKSTEGKSSGSGSESKSTGGGGSQIQLQQSGPEVVKPGASVKISCKASGYTFISYYIHWVKQRPGQGLEWIGWIYPGDGSTNNNEKFKGKTTLTADKSSSTAYMLLSSLTSEDSAVYFCARGEGNAMDDWGQGTSVTVSSASTKGPSVFPLAPSSKSTSGGTAALGCLVKDYFPEPVTVSWNSGALTSGVHTFPAVLQSSGLYSLSSVVTVPSSSLGTQTYICNVNHKPSNTKVDKRVEPKSCDKTHTCPPCPAPEAAGGPSVFLFPPKPKDTLMISRTPEVTCVVVDVSHEDPEVKFNWYVDGVEVHNAKTKPREEQYNSTYRVVSVLTVLHQDWLNGKEYKCKVSNKALPAPIEKTISKAKGQPREPQVYTLPPSREEMTKNQVSLWCLVKGFYPSDIAVEWESNGQPENNYKTTPPVLDSDGSFFLYSKLTVDKSRWQQGNVFSCSVMHEALHNHYTQKSLSLSPG

SEQ ID NO: 252 - protein, 698 aa, Artificial Sequence
  DLL3#18 chain
DIQMTQSPASLAASVGETVTITCRASENIYYSLAWYQQKQGKSPQLLIYNANSLEDGVPSRFSGSGSGTQYSMKINNMQPEDTATYFCKQAYDVPLTFGAGTKLELKRTVAAPSVFIFPPSDEQLKSGTASVVCLLNNFYPREAKVQWKVDNALQSGNSQESVTEQDSKDSTYSLSSTLTLSKADYEKHKVYACEVTHQGLSSPVTKSFNRGECGGGGSEGKSSGSGSESKSTEGKSSGSGSESKSTGGGGSQVQLQQSGPDLVKPGASVKMSCEASGYTFTAYFIHWVKQKPGQGLEWIGYIDPFNDDTNYNVKFKGKATLTSDTSSSIAYMELSSLTSEDSSFYYCARGTSATLDYWGHGTTLTVSSASTKGPSVFPLAPSSKSTSGGTAALGCLVKDYFPEPVTVSWNSGALTSGVHTFPAVLQSSGLYSLSSVVTVPSSSLGTQTYICNVNHKPSNTKVDKRVEPKSCDKTHTCPPCPAPEAAGGPSVFLFPPKPKDTLMISRTPEVTCVVVDVSHEDPEVKFNWYVDGVEVHNAKTKPREEQYNSTYRVVSVLTVLHQDWLNGKEYKCKVSNKALPAPIEKTISKAKGQPREPQVYTLPPSREEMTKNQVSLWCLVKGFYPSDIAVEWESNGQPENNYKTTPPVLDSDGSFFLYSKLTVDKSRWQQGNVFSCSVMHEALHNHYTQKSLSLSPG

SEQ ID NO: 253 - protein, 61 aa, Artificial Sequence
  region of heavy chain
SGALTSGVHTFPAVLQSSGLYSLSSVVTVPSSSLGTQTYICNVNHKPSNTKVDKRVEPKSC

SEQ ID NO: 254 - protein, 330 aa, Artificial Sequence
  Mouse
AKTTAPSVYPLAPVCGDTTGSSVTLGCLVKGYFPEPVTLTWNSGSLSSGVHTFPAVLQSDLYTLSSSVTVTSSTWPSQSITCNVAHPASSTKVDKKIEPRGPTIKPCPPCKCPAPNLLGGPSVFIFPPKIKDVLMISLSPIVTCVVVDVSEDDPDVQISWFVNNVEVHTAQTQTHREDYNSTLRVVSALPIQHQDWMSGKEFKCKVNNKDLPAPIERTISKPKGSVRAPQVYVLPPPEEEMTKKQVTLTCMVTDFMPEDIYVEWTNNGKTELNYKNTEPVLDSDGSYFMYSKLRVEKKNWVERNSYSCSVVHEGLHNHHTTKSFSRTPGK

SEQ ID NO: 255 - protein, 107 aa, Artificial Sequence
  Mouse
RADAAPTVSIFPPSSEQLTSGGASVVCFLNNFYPKDINVKWKIDGSERQNGVLNSWTDQDSKDSTYSMSSTLTLTKDEYERHNSYTCEATHKTSTSPIVKSFNRNEC

SEQ ID NO: 256 - protein, 446 aa, Artificial Sequence
  PD1-1 HC
EVMLVESGGGLVQPGGSLRLSCTASGFTFSASAMSWVRQAPGKGLEWVAYISGGGGDTYYSSSVKGRFTISRDNAKNSLYLQMNSLRAEDTAVYYCARHSNVNYYAMDYWGQGTLVTVSSASTKGPSVFPLAPCSRSTSESTAALGCLVKDYFPEPVTVSWNSGALTSGVHTFPAVLQSSGLYSLSSVVTVPSSSLGTKTYTCNVDHKPSNTKVDKRVESKYGPPCPPCPAPEFLGGPSVFLFPPKPKDTLMISRTPEVTCVVVDVSQEDPEVQFNWYVDGVEVHNAKTKPREEQFNSTYRVVSVLTVLHQDWLNGKEYKCKVSNKGLPSSIEKTISKAKGQPREPQVYTLPPSQEEMTKNQVSLTCLVKGFYPSDIAVEWESNGQPENNYKTTPPVLDSDGSFFLYSRLTVDKSRWQEGNVFSCSVMHEALHNHYTQKSLSLSLG

SEQ ID NO: 257 - protein, 218 aa, Artificial Sequence
  PD1-1 LC
EIVLTQSPATLSLSPGERATMSCRASENIDTSGISFMNWYQQKPGQAPKLLIYVASNQGSGIPARFSGSGSGTDFTLTISRLEPEDFAVYYCQQSKEVPWTFGQGTKLEIKRTVAAPSVFIFPPSDEQLKSGTASVVCLLNNFYPREAKVQWKVDNALQSGNSQESVTEQDSKDSTYSLSSTLTLSKADYEKHKVYACEVTHQGLSSPVTKSFNRGEC

SEQ ID NO: 258 - protein, 446 aa, Artificial Sequence
  PD1-2 HC
EVMLVESGGGLVQPGGSLRLSCTASGFTFSASAMSWVRQAPGKGLEWVAYISGGGGDTYYSSSVKGRFTISRDNAKNSLYLQMNSLRAEDTAVYYCARHSNPNYYAMDYWGQGTLVTVSSASTKGPSVFPLAPCSRSTSESTAALGCLVKDYFPEPVTVSWNSGALTSGVHTFPAVLQSSGLYSLSSVVTVPSSSLGTKTYTCNVDHKPSNTKVDKRVESKYGPPCPPCPAPEFLGGPSVFLFPPKPKDTLMISRTPEVTCVVVDVSQEDPEVQFNWYVDGVEVHNAKTKPREEQFNSTYRVVSVLTVLHQDWLNGKEYKCKVSNKGLPSSIEKTISKAKGQPREPQVYTLPPSQEEMTKNQVSLTCLVKGFYPSDIAVEWESNGQPENNYKTTPPVLDSDGSFFLYSRLTVDKSRWQEGNVFSCSVMHEALHNHYTQKSLSLSLG

SEQ ID NO: 259 - protein, 218 aa, Artificial Sequence; identical to SEQ ID NO: 257
  PD1-2 LC

SEQ ID NO: 260 - protein, 446 aa, Artificial Sequence
  PD1-3 HC
EVMLVESGGGLVQPGGSLRLSCTASGFTFSKSAMSWVRQAPGKGLEWVAYISGGGGDTYYSSSVKGRFTISRDNAKNSLYLQMNSLRAEDTAVYYCARHSNVNYYAMDYWGQGTLVTVSSASTKGPSVFPLAPCSRSTSESTAALGCLVKDYFPEPVTVSWNSGALTSGVHTFPAVLQSSGLYSLSSVVTVPSSSLGTKTYTCNVDHKPSNTKVDKRVESKYGPPCPPCPAPEFLGGPSVFLFPPKPKDTLMISRTPEVTCVVVDVSQEDPEVQFNWYVDGVEVHNAKTKPREEQFNSTYRVVSVLTVLHQDWLNGKEYKCKVSNKGLPSSIEKTISKAKGQPREPQVYTLPPSQEEMTKNQVSLTCLVKGFYPSDIAVEWESNGQPENNYKTTPPVLDSDGSFFLYSRLTVDKSRWQEGNVFSCSVMHEALHNHYTQKSLSLSLG

SEQ ID NO: 261 - protein, 218 aa, Artificial Sequence
  PD1-3 LC
EIVLTQSPATLSLSPGERATMSCRASENIDVSGISFMNWYQQKPGQAPKLLIYVASNQGSGIPARFSGSGSGTDFTLTISRLEPEDFAVYYCQQSKEVPWTFGQGTKLEIKRTVAAPSVFIFPPSDEQLKSGTASVVCLLNNFYPREAKVQWKVDNALQSGNSQESVTEQDSKDSTYSLSSTLTLSKADYEKHKVYACEVTHQGLSSPVTKSFNRGEC

SEQ ID NO: 262 - protein, 446 aa, Artificial Sequence; identical to SEQ ID NO: 260
  PD1-4 HC

SEQ ID NO: 263 - protein, 218 aa, Artificial Sequence; identical to SEQ ID NO: 261
  PD1-4 LC

SEQ ID NO: 264 - protein, 446 aa, Artificial Sequence; identical to SEQ ID NO: 260
  PD1-5 HC

SEQ ID NO: 265 - protein, 218 aa, Artificial Sequence; identical to SEQ ID NO: 261
  PD1-5 LC